European Patent Specification EP 3 638 700 B1, published July 24, 2024. Title: PROTEINACEOUS HETERODIMER AND USE THEREOF. Applicant: Dingfu Biotarget Co., Ltd. The sequence listing filed with the application follows.

SEQUENCE LISTING (180 sequences)

SEQ ID NO: 1 - protein, 227 aa, Artificial Sequence
  A Y349C+T366W
DKTHTCPPCPAPELLGGPSVFLFPPKPKDTLMISRTPEVTCVVVDVSHENPEVKFNWYVDGVEVHNAKTKPREEQYNSTYRVVSVLTVLHQDWLNGKEYKCKVSNKALPAPIEKTISKAKGQPREPQVCTLPPSRDELTKNQVSLWCLVKGFYPSDIAVEWESNGQPENNYKTTPPVLDSDGSFFLYSKLTVDKSRWQQGNVFSCSVMHEALHNHYTQKSLSLSPGK

SEQ ID NO: 2 - protein, 227 aa, Artificial Sequence
  B D356C+T366S+L368A+Y407V
DKTHTCPPCPAPELLGGPSVFLFPPKPKDTLMISRTPEVTCVVVDVSHEDPEVKFNWYVDGVEVHNAKTKPREEQYNSTYRVVSVLTVLHQDWLNGKEYKCKVSNKALPAPIEKTISKAKGQPREPQVYTLPPSRCELTKNQVSLSCAVKGFYPSDIAVEWESNGQPENNYKTTPPVLDSDGSFFLVSKLTVDKSRWQQGNVFSCSVMHEALHNHYTQKSLSLSPGK

SEQ ID NO: 3 - protein, 227 aa, Artificial Sequence
  B D356C+T366S+L368A+Y407V+F405K
DKTHTCPPCPAPELLGGPSVFLFPPKPKDTLMISRTPEVTCVVVDVSHEDPEVKFNWYVDGVEVHNAKTKPREEQYNSTYRVVSVLTVLHQDWLNGKEYKCKVSNKALPAPIEKTISKAKGQPREPQVYTLPPSRCELTKNQVSLSCAVKGFYPSDIAVEWESNGQPENNYKTTPPVLDSDGSFKLVSKLTVDKSRWQQGNVFSCSVMHEALHNHYTQKSLSLSPGK

SEQ ID NO: 4 - protein, 227 aa, Artificial Sequence
  A Y349C+T366W+F405K
DKTHTCPPCPAPELLGGPSVFLFPPKPKDTLMISRTPEVTCVVVDVSHENPEVKFNWYVDGVEVHNAKTKPREEQYNSTYRVVSVLTVLHQDWLNGKEYKCKVSNKALPAPIEKTISKAKGQPREPQVCTLPPSRDELTKNQVSLWCLVKGFYPSDIAVEWESNGQPENNYKTTPPVLDSDGSFKLYSKLTVDKSRWQQGNVFSCSVMHEALHNHYTQKSLSLSPGK

SEQ ID NO: 5 - protein, 227 aa, Artificial Sequence
  A Y349C+T366W+K409E
DKTHTCPPCPAPELLGGPSVFLFPPKPKDTLMISRTPEVTCVVVDVSHENPEVKFNWYVDGVEVHNAKTKPREEQYNSTYRVVSVLTVLHQDWLNGKEYKCKVSNKALPAPIEKTISKAKGQPREPQVCTLPPSRDELTKNQVSLWCLVKGFYPSDIAVEWESNGQPENNYKTTPPVLDSDGSFFLYSELTVDKSRWQQGNVFSCSVMHEALHNHYTQKSLSLSPGK

SEQ ID NO: 6 - protein, 227 aa, Artificial Sequence
  A Y349C+T366W+K409A
DKTHTCPPCPAPELLGGPSVFLFPPKPKDTLMISRTPEVTCVVVDVSHENPEVKFNWYVDGVEVHNAKTKPREEQYNSTYRVVSVLTVLHQDWLNGKEYKCKVSNKALPAPIEKTISKAKGQPREPQVCTLPPSRDELTKNQVSLWCLVKGFYPSDIAVEWESNGQPENNYKTTPPVLDSDGSFFLYSALTVDKSRWQQGNVFSCSVMHEALHNHYTQKSLSLSPGK

SEQ ID NO: 7 - protein, 227 aa, Artificial Sequence
  A Y349C+T366W+F405K+K360E+Q347E
DKTHTCPPCPAPELLGGPSVFLFPPKPKDTLMISRTPEVTCVVVDVSHENPEVKFNWYVDGVEVHNAKTKPREEQYNSTYRVVSVLTVLHQDWLNGKEYKCKVSNKALPAPIEKTISKAKGQPREPEVCTLPPSRDELTENQVSLWCLVKGFYPSDIAVEWESNGQPENNYKTTPPVLDSDGSFKLYSKLTVDKSRWQQGNVFSCSVMHEALHNHYTQKSLSLSPGK

SEQ ID NO: 8 - protein, 227 aa, Artificial Sequence
  B D356C+T366S+L368A+Y407V+Q347R
DKTHTCPPCPAPELLGGPSVFLFPPKPKDTLMISRTPEVTCVVVDVSHEDPEVKFNWYVDGVEVHNAKTKPREEQYNSTYRVVSVLTVLHQDWLNGKEYKCKVSNKALPAPIEKTISKAKGQPREPRVYTLPPSRCELTKNQVSLSCAVKGFYPSDIAVEWESNGQPENNYKTTPPVLDSDGSFFLVSKLTVDKSRWQQGNVFSCSVMHEALHNHYTQKSLSLSPGK

SEQ ID NO: 9 - protein, 227 aa, Artificial Sequence
  A Y349C+T366W+F405K+Q347R
DKTHTCPPCPAPELLGGPSVFLFPPKPKDTLMISRTPEVTCVVVDVSHENPEVKFNWYVDGVEVHNAKTKPREEQYNSTYRVVSVLTVLHQDWLNGKEYKCKVSNKALPAPIEKTISKAKGQPREPRVCTLPPSRDELTKNQVSLWCLVKGFYPSDIAVEWESNGQPENNYKTTPPVLDSDGSFKLYSKLTVDKSRWQQGNVFSCSVMHEALHNHYTQKSLSLSPGK

SEQ ID NO: 10 - protein, 227 aa, Artificial Sequence
  B D356C+T366S+L368A+Y407V+K360E+Q347E
DKTHTCPPCPAPELLGGPSVFLFPPKPKDTLMISRTPEVTCVVVDVSHEDPEVKFNWYVDGVEVHNAKTKPREEQYNSTYRVVSVLTVLHQDWLNGKEYKCKVSNKALPAPIEKTISKAKGQPREPEVYTLPPSRCELTENQVSLSCAVKGFYPSDIAVEWESNGQPENNYKTTPPVLDSDGSFFLVSKLTVDKSRWQQGNVFSCSVMHEALHNHYTQKSLSLSPGK

SEQ ID NO: 11 - protein, 227 aa, Artificial Sequence
  A Y349C+T366W+K409A+K360E+Q347E
DKTHTCPPCPAPELLGGPSVFLFPPKPKDTLMISRTPEVTCVVVDVSHENPEVKFNWYVDGVEVHNAKTKPREEQYNSTYRVVSVLTVLHQDWLNGKEYKCKVSNKALPAPIEKTISKAKGQPREPEVCTLPPSRDELTENQVSLWCLVKGFYPSDIAVEWESNGQPENNYKTTPPVLDSDGSFFLYSALTVDKSRWQQGNVFSCSVMHEALHNHYTQKSLSLSPGK

SEQ ID NO: 12 - protein, 227 aa, Artificial Sequence
  B D356C+T366S+L368A+Y407V+F405K+Q347R
DKTHTCPPCPAPELLGGPSVFLFPPKPKDTLMISRTPEVTCVVVDVSHEDPEVKFNWYVDGVEVHNAKTKPREEQYNSTYRVVSVLTVLHQDWLNGKEYKCKVSNKALPAPIEKTISKAKGQPREPRVYTLPPSRCELTKNQVSLSCAVKGFYPSDIAVEWESNGQPENNYKTTPPVLDSDGSFKLVSKLTVDKSRWQQGNVFSCSVMHEALHNHYTQKSLSLSPGK

SEQ ID NO: 13 - protein, 227 aa, Artificial Sequence
  A Y349C+T366W+K409A+Q347R
DKTHTCPPCPAPELLGGPSVFLFPPKPKDTLMISRTPEVTCVVVDVSHENPEVKFNWYVDGVEVHNAKTKPREEQYNSTYRVVSVLTVLHQDWLNGKEYKCKVSNKALPAPIEKTISKAKGQPREPRVCTLPPSRDELTKNQVSLWCLVKGFYPSDIAVEWESNGQPENNYKTTPPVLDSDGSFFLYSALTVDKSRWQQGNVFSCSVMHEALHNHYTQKSLSLSPGK

SEQ ID NO: 14 - protein, 227 aa, Artificial Sequence
  B D356C+T366S+L368A+Y407V+F405K+K360E+Q347E
DKTHTCPPCPAPELLGGPSVFLFPPKPKDTLMISRTPEVTCVVVDVSHEDPEVKFNWYVDGVEVHNAKTKPREEQYNSTYRVVSVLTVLHQDWLNGKEYKCKVSNKALPAPIEKTISKAKGQPREPEVYTLPPSRCELTENQVSLSCAVKGFYPSDIAVEWESNGQPENNYKTTPPVLDSDGSFKLVSKLTVDKSRWQQGNVFSCSVMHEALHNHYTQKSLSLSPGK

SEQ ID NO: 15 - protein, 227 aa, Artificial Sequence
  A T366W+K409A+K392D
DKTHTCPPCPAPELLGGPSVFLFPPKPKDTLMISRTPEVTCVVVDVSHENPEVKFNWYVDGVEVHNAKTKPREEQYNSTYRVVSVLTVLHQDWLNGKEYKCKVSNKALPAPIEKTISKAKGQPREPQVYTLPPSRDELTKNQVSLWCLVKGFYPSDIAVEWESNGQPENNYDTTPPVLDSDGSFFLYSALTVDKSRWQQGNVFSCSVMHEALHNHYTQKSLSLSPGK

SEQ ID NO: 16 - protein, 227 aa, Artificial Sequence
  B T366S+L368A+Y407V+D399S+F405K
DKTHTCPPCPAPELLGGPSVFLFPPKPKDTLMISRTPEVTCVVVDVSHEDPEVKFNWYVDGVEVHNAKTKPREEQYNSTYRVVSVLTVLHQDWLNGKEYKCKVSNKALPAPIEKTISKAKGQPREPQVYTLPPSRDELTKNQVSLSCAVKGFYPSDIAVEWESNGQPENNYKTTPPVLSSDGSFKLVSKLTVDKSRWQQGNVFSCSVMHEALHNHYTQKSLSLSPGK

SEQ ID NO: 17 - protein, 227 aa, Artificial Sequence
  A T366W+K409A
DKTHTCPPCPAPELLGGPSVFLFPPKPKDTLMISRTPEVTCVVVDVSHENPEVKFNWYVDGVEVHNAKTKPREEQYNSTYRVVSVLTVLHQDWLNGKEYKCKVSNKALPAPIEKTISKAKGQPREPQVYTLPPSRDELTKNQVSLWCLVKGFYPSDIAVEWESNGQPENNYKTTPPVLDSDGSFFLYSALTVDKSRWQQGNVFSCSVMHEALHNHYTQKSLSLSPGK

SEQ ID NO: 18 - protein, 227 aa, Artificial Sequence
  B T366S+L368G+Y407A+F405K
DKTHTCPPCPAPELLGGPSVFLFPPKPKDTLMISRTPEVTCVVVDVSHEDPEVKFNWYVDGVEVHNAKTKPREEQYNSTYRVVSVLTVLHQDWLNGKEYKCKVSNKALPAPIEKTISKAKGQPREPQVYTLPPSRDELTKNQVSLSCGVKGFYPSDIAVEWESNGQPENNYKTTPPVLDSDGSFKLASKLTVDKSRWQQGNVFSCSVMHEALHNHYTQKSLSLSPGK

SEQ ID NO: 19 - protein, 227 aa, Artificial Sequence
  A T366W+K409A+Y349D
DKTHTCPPCPAPELLGGPSVFLFPPKPKDTLMISRTPEVTCVVVDVSHENPEVKFNWYVDGVEVHNAKTKPREEQYNSTYRVVSVLTVLHQDWLNGKEYKCKVSNKALPAPIEKTISKAKGQPREPQVDTLPPSRDELTKNQVSLWCLVKGFYPSDIAVEWESNGQPENNYKTTPPVLDSDGSFFLYSALTVDKSRWQQGNVFSCSVMHEALHNHYTQKSLSLSPGK

SEQ ID NO: 20 - protein, 227 aa, Artificial Sequence
  B T366S+L368A+Y407V+F405K+E357A
DKTHTCPPCPAPELLGGPSVFLFPPKPKDTLMISRTPEVTCVVVDVSHEDPEVKFNWYVDGVEVHNAKTKPREEQYNSTYRVVSVLTVLHQDWLNGKEYKCKVSNKALPAPIEKTISKAKGQPREPQVYTLPPSRDALTKNQVSLSCAVKGFYPSDIAVEWESNGQPENNYKTTPPVLDSDGSFKLVSKLTVDKSRWQQGNVFSCSVMHEALHNHYTQKSLSLSPGK

SEQ ID NO: 21 - protein, 227 aa, Artificial Sequence
  A T366W+K409A+Y349D+S354D
DKTHTCPPCPAPELLGGPSVFLFPPKPKDTLMISRTPEVTCVVVDVSHENPEVKFNWYVDGVEVHNAKTKPREEQYNSTYRVVSVLTVLHQDWLNGKEYKCKVSNKALPAPIEKTISKAKGQPREPQVDTLPPDRDELTKNQVSLWCLVKGFYPSDIAVEWESNGQPENNYKTTPPVLDSDGSFFLYSALTVDKSRWQQGNVFSCSVMHEALHNHYTQKSLSLSPGK

SEQ ID NO: 22 - protein, 227 aa, Artificial Sequence
  A T366W+F405K
DKTHTCPPCPAPELLGGPSVFLFPPKPKDTLMISRTPEVTCVVVDVSHENPEVKFNWYVDGVEVHNAKTKPREEQYNSTYRVVSVLTVLHQDWLNGKEYKCKVSNKALPAPIEKTISKAKGQPREPQVYTLPPSRDELTKNQVSLWCLVKGFYPSDIAVEWESNGQPENNYKTTPPVLDSDGSFKLYSKLTVDKSRWQQGNVFSCSVMHEALHNHYTQKSLSLSPGK

SEQ ID NO: 23 - protein, 227 aa, Artificial Sequence
  B T366S+L368A+Y407V+K409A
DKTHTCPPCPAPELLGGPSVFLFPPKPKDTLMISRTPEVTCVVVDVSHEDPEVKFNWYVDGVEVHNAKTKPREEQYNSTYRVVSVLTVLHQDWLNGKEYKCKVSNKALPAPIEKTISKAKGQPREPQVYTLPPSRDELTKNQVSLSCAVKGFYPSDIAVEWESNGQPENNYKTTPPVLDSDGSFFLVSALTVDKSRWQQGNVFSCSVMHEALHNHYTQKSLSLSPGK

SEQ ID NO: 24 - protein, 227 aa, Artificial Sequence
  A T366W+F405K+D399S
DKTHTCPPCPAPELLGGPSVFLFPPKPKDTLMISRTPEVTCVVVDVSHENPEVKFNWYVDGVEVHNAKTKPREEQYNSTYRVVSVLTVLHQDWLNGKEYKCKVSNKALPAPIEKTISKAKGQPREPQVYTLPPSRDELTKNQVSLWCLVKGFYPSDIAVEWESNGQPENNYKTTPPVLSSDGSFKLYSKLTVDKSRWQQGNVFSCSVMHEALHNHYTQKSLSLSPGK

SEQ ID NO: 25 - protein, 227 aa, Artificial Sequence
  B T366S+L368A+Y407V+K409A+K392D
DKTHTCPPCPAPELLGGPSVFLFPPKPKDTLMISRTPEVTCVVVDVSHEDPEVKFNWYVDGVEVHNAKTKPREEQYNSTYRVVSVLTVLHQDWLNGKEYKCKVSNKALPAPIEKTISKAKGQPREPQVYTLPPSRDELTKNQVSLSCAVKGFYPSDIAVEWESNGQPENNYDTTPPVLDSDGSFFLVSALTVDKSRWQQGNVFSCSVMHEALHNHYTQKSLSLSPGK

SEQ ID NO: 26 - protein, 227 aa, Artificial Sequence
  A T366S+L368G+Y407A+K409A
DKTHTCPPCPAPELLGGPSVFLFPPKPKDTLMISRTPEVTCVVVDVSHEDPEVKFNWYVDGVEVHNAKTKPREEQYNSTYRVVSVLTVLHQDWLNGKEYKCKVSNKALPAPIEKTISKAKGQPREPQVYTLPPSRDELTKNQVSLSCGVKGFYPSDIAVEWESNGQPENNYKTTPPVLDSDGSFFLASALTVDKSRWQQGNVFSCSVMHEALHNHYTQKSLSLSPGK

SEQ ID NO: 27 - protein, 227 aa, Artificial Sequence
  A T366W +F405K +Y349D
DKTHTCPPCPAPELLGGPSVFLFPPKPKDTLMISRTPEVTCVVVDVSHENPEVKFNWYVDGVEVHNAKTKPREEQYNSTYRVVSVLTVLHQDWLNGKEYKCKVSNKALPAPIEKTISKAKGQPREPQVDTLPPSRDELTKNQVSLWCLVKGFYPSDIAVEWESNGQPENNYKTTPPVLDSDGSFKLYSKLTVDKSRWQQGNVFSCSVMHEALHNHYTQKSLSLSPGK

SEQ ID NO: 28 - protein, 227 aa, Artificial Sequence
  B T366S+L368A+Y407V +K409A +E357A
DKTHTCPPCPAPELLGGPSVFLFPPKPKDTLMISRTPEVTCVVVDVSHEDPEVKFNWYVDGVEVHNAKTKPREEQYNSTYRVVSVLTVLHQDWLNGKEYKCKVSNKALPAPIEKTISKAKGQPREPQVYTLPPSRDALTKNQVSLSCAVKGFYPSDIAVEWESNGQPENNYKTTPPVLDSDGSFFLVSALTVDKSRWQQGNVFSCSVMHEALHNHYTQKSLSLSPGK

SEQ ID NO: 29 - protein, 227 aa, Artificial Sequence
  A T366W+F405K+Y349D+S354D
DKTHTCPPCPAPELLGGPSVFLFPPKPKDTLMISRTPEVTCVVVDVSHENPEVKFNWYVDGVEVHNAKTKPREEQYNSTYRVVSVLTVLHQDWLNGKEYKCKVSNKALPAPIEKTISKAKGQPREPQVDTLPPDRDELTKNQVSLWCLVKGFYPSDIAVEWESNGQPENNYKTTPPVLDSDGSFKLYSKLTVDKSRWQQGNVFSCSVMHEALHNHYTQKSLSLSPGK

SEQ ID NO: 30 - protein, 227 aa, Homo sapiens
DKTHTCPPCPAPELLGGPSVFLFPPKPKDTLMISRTPEVTCVVVDVSHEDPEVKFNWYVDGVEVHNAKTKPREEQYNSTYRVVSVLTVLHQDWLNGKEYKCKVSNKALPAPIEKTISKAKGQPREPQVYTLPPSRDELTKNQVSLTCLVKGFYPSDIAVEWESNGQPENNYKTTPPVLDSDGSFFLYSKLTVDKSRWQQGNVFSCSVMHEALHNHYTQKSLSLSPGK

SEQ ID NO: 31 - DNA, 681 bp, Homo sapiens
gacaagacccacacctgccccccctgccccgcccccgagctgctgggcggccccagcgtgttcctgttcccccccaagcccaaggacaccctgatgatcagccgcacccccgaggtgacctgcgtggtggtggacgtgagccacgagaaccccgaggtgaagttcaactggtacgtggacggcgtggaggtgcacaacgccaagaccaagccccgcgaggagcagtacaacagcacctaccgcgtggtgagcgtgctgaccgtgctgcaccaggactggctgaacggcaaggagtacaagtgcaaggtgagcaacaaggccctgcccgcccccatcgagaagaccatcagcaaggccaagggccagccccgcgagccccaggtgtacaccctgccccccagccgcgacgagctgaccaagaaccaggtgagcctgacctgcctggtgaagggcttctaccccagcgacatcgccgtggagtgggagagcaacggccagcccgagaacaactacaagaccaccccccccgtgctggacagcgacggcagcttcttcctgtacagcaagctgaccgtggacaagagccgctggcagcagggcaacgtgttcagctgcagcgtgatgcacgaggccctgcacaaccactacacccagaagagcctgagcctgagccccggcaag

SEQ ID NO: 32 - DNA, 741 bp, Mus musculus
atggagaccgacaccctgctgctgtgggtgctgctgctgtgggtgcccggcagcaccggcgacaagacccacacctgccccccctgccccgcccccgagctgctgggcggccccagcgtgttcctgttcccccccaagcccaaggacaccctgatgatcagccgcacccccgaggtgacctgcgtggtggtggacgtgagccacgagaaccccgaggtgaagttcaactggtacgtggacggcgtggaggtgcacaacgccaagaccaagccccgcgaggagcagtacaacagcacctaccgcgtggtgagcgtgctgaccgtgctgcaccaggactggctgaacggcaaggagtacaagtgcaaggtgagcaacaaggccctgcccgcccccatcgagaagaccatcagcaaggccaagggccagccccgcgagccccaggtgtacaccctgccccccagccgcgacgagctgaccaagaaccaggtgagcctgacctgcctggtgaagggcttctaccccagcgacatcgccgtggagtgggagagcaacggccagcccgagaacaactacaagaccaccccccccgtgctggacagcgacggcagcttcttcctgtacagcaagctgaccgtggacaagagccgctggcagcagggcaacgtgttcagctgcagcgtgatgcacgaggccctgcacaaccactacacccagaagagcctgagcctgagccccggcaag

SEQ ID NO: 33 - DNA, 1121 bp, Artificial Sequence
  fusion gene fragment
atggagaccgacaccctgctgctgtgggtgctgctgctgtgggtgcccggcagcaccggccaggtgcagctgcaggagtctgggggaggctcggtgcaggctggagggtctctgagactctcctgtgcagcctctgaatacatctacagtagctactgcatggcctggttccgccaggctccagggaaggagcgcgagggggtcgcagttattgggagtgatggtagcacaagctacgcagactccgtgaaaggccgattcaccatctccaaagacaacgccaagaacactctgtatctgcaaatgaacagcctgaaacctgaggacactgccatgtactactgtgcggccatcggtggttactgctaccaaccaccctatgagtaccagtactggggccaggggacccaggtcaccgtctcccagaaccgaaaagcagcgacaagacccacacctgccccccctgccccgcccccgagctgctgggcggccccagcgtgttcctgttcccccccaagcccaaggacaccctgatgatcagccgcacccccgaggtgacctgcgtggtggtggacgtgagccacgagaaccccgaggtgaagttcaactggtacgtggacggcgtggaggtgcacaacgccaagaccaagccccgcgaggagcagtacaacagcacctaccgcgtggtgagcgtgctgaccgtgctgcaccaggactggctgaacggcaaggagtacaagtgcaaggtgagcaacaaggccctgcccgcccccatcgagaagaccatcagcaaggccaagggccagccccgcgagccccaggtgtacaccctgccccccagccgcgacgagctgaccaagaaccaggtgagcctgacctgcctggtgaagggcttctaccccagcgacatcgccgtggagtgggagagcaacggccagcccgagaacaactacaagaccaccccccccgtgctggacagcgacggcagcttcttcctgtacagcaagctgaccgtggacaagagccgctggcagcagggcaacgtgttcagctgcagcgtgatgcacgaggccctgcacaaccactacacccagaagagcctgagcctgagccccggcaag

SEQ ID NO: 34 - protein, 354 aa, Artificial Sequence
  fusion protein VhH-Fc
QVQLQESGGGSVQAGGSLRLSCAASEYIYSSYCMAWFRQAPGKEREGVAVIGSDGSTSYADSVKGRFTISKDNAKNTLYLQMNSLKPEDTAMYYCAAIGGYCYQPPYEYQYWGQGTQVTVSSEPKSSDKTHTCPPCPAPELLGGPSVFLFPPKPKDTLMISRTPEVTCVVVDVSHEDPEVKFNWYVDGVEVHNAKTKPREEQYNSTYRVVSVLTVLHQDWLNGKEYKCKVSNKALPAPIEKTISKAKGQPREPQVYTLPPSRDELTKNQVSLTCLVKGFYPSDIAVEWESNGQPENNYKTTPPVLDSDGSFFLYSKLTVDKSRWQQGNVFSCSVMHEALHNHYTQKSLSLSPGK

SEQ ID NO: 35 - DNA, 1473 bp, Artificial Sequence
  gene for anti-Her2 single chain ScFv-Fc fusion protein
atggagaccgacaccctgctgctgtgggtgctgctgctgtgggtgcccggcagcaccggcgaggtgcagctgctggagagcggcggcggcgtggtgcagcccggccgcagcctgcgcctgagctgcatcgccagcggcttcaccttcagcagctaccccatgacctgggtgcgccaggcccccggcaagggcctggagtgggtggccagcatcagctacgacggcagctacaagtacaaggccgacagcatgaagggccgcctgaccatcagccgcgacaacagcaagaacaccctgtacctggagatgaacagcctgaccgccgaggacaccgccgtgtactactgcgcccgcaccgccttcttcaacgcctacgacttctggggccagggcaccctggtgaccgtgagcagcgccagcaccaagggccccagcgtgggcggcggcggcagcggcggcggcggcagcgagatcgtgatgacccagagccccgccaccctgagcgtgagccccggcgagcgcgccaccctgagctgccgcgccagccagagcgtgcgcagcaacctggcctggtaccagcagaagcccggccaggccccccgcctgctgatctacgccgccagcacccgcgccaccggcatccccgcccgcttcagcggcagcggcagcggcaccgagttcaccctgaccatcagcagcctgcagagcgaggacttcgccgtgtactactgccagcagtacaacgagtggttccgcaccagcggccagggcaccaaggtggagatcaagcgcgacaagacccacacctgccccccctgccccgcccccgagctgctgggcggccccagcgtgttcctgttcccccccaagcccaaggacaccctgatgatcagccgcacccccgaggtgacctgcgtggtggtggacgtgagccacgagaaccccgaggtgaagttcaactggtacgtggacggcgtggaggtgcacaacgccaagaccaagccccgcgaggagcagtacaacagcacctaccgcgtggtgagcgtgctgaccgtgctgcaccaggactggctgaacggcaaggagtacaagtgcaaggtgagcaacaaggccctgcccgcccccatcgagaagaccatcagcaaggccaagggccagccccgcgagccccaggtgtacaccctgccccccagccgcgacgagctgaccaagaaccaggtgagcctgacctgcctggtgaagggcttctaccccagcgacatcgccgtggagtgggagagcaacggccagcccgagaacaactacaagaccaccccccccgtgctggacagcgacggcagcttcttcctgtacagcaagctgaccgtggacaagagccgctggcagcagggcaacgtgttcagctgcagcgtgatgcacgaggccctgcacaaccactacacccagaagagcctgagcctgagccccggcaag

SEQ ID NO: 36 - protein, 471 aa, Artificial Sequence
  anti-Her2 single chain ScFv -Fc fusion protein
EVQLLESGGGVVQPGRSLRLSCIASGFTFSSYPMTWVRQAPGKGLEWVASISYDGSYKYKADSMKGRLTISRDNSKNTLYLEMNSLTAEDTAVYYCARTAFFNAYDFWGQGTLVTVSSASTKGPSVGGGGSGGGGSEIVMTQSPATLSVSPGERATLSCRASQSVRSNLAWYQQKPGQAPRLLIYAASTRATGIPARFSGSGSGTEFTLTISSLQSEDFAVYYCQQYNEWFRTSGQGTKVEIKRDKTHTCPPCPAPELLGGPSVFLFPPKPKDTLMISRTPEVTCVVVDVSHENPEVKFNWYVDGVEVHNAKTKPREEQYNSTYRVVSVLTVLHQDWLNGKEYKCKVSNKALPAPIEKTISKAKGQPREPQVYTLPPSRDELTKNQVSLTCLVKGFYPSDIAVEWESNGQPENNYKTTPPVLDSDGSFFLYSKLTVDKSRWQQGNVFSCSVMHEALHNHYTQKSLSLSPGK

SEQ ID NO: 37 - protein, 214 aa, Artificial Sequence
  Erb-LC
DILLTQSPVILSVSPGERVSFSCRASQSIGTNIHWYQQRTNGSPRLLIKYASESISGIPSRFSGSGSGTDFTLSINSVESEDIADYYCQQNNNWPTTFGAGTKLELKRTVAAPSVFIFPPSDEQLKSGTASVVCLLNNFYPREAKVQWKVDNALQSGNSQESVTEQDSKDSTYSLSSTLTLSKADYEKHKVYACEVTHQGLSSPVTKSFNRGEC

SEQ ID NO: 38 - DNA, 642 bp, Artificial Sequence
  nucleic acid molecules encoding Erb-LC
gacatcctgctgacccagagccccgtgatcctgagcgtgagccccggcgagcgcgtgagcttcagctgccgcgccagccagagcatcggcaccaacatccactggtaccagcagcgcaccaacggcagcccccgcctgctgatcaagtacgccagcgagagcatcagcggcatccccagccgcttcagcggcagcggcagcggcaccgacttcaccctgagcatcaacagcgtggagagcgaggacatcgccgactactactgccagcagaacaacaactggcccaccaccttcggcgccggcaccaagctggagctgaagcgcaccgtggccgcccccagcgtgttcatcttcccccccagcgacgagcagctgaagagcggcaccgccagcgtggtgtgcctgctgaacaacttctacccccgcgaggccaaggtgcagtggaaggtggacaacgccctgcagagcggcaacagccaggagagcgtgaccgagcaggacagcaaggacagcacctacagcctgagcagcaccctgaccctgagcaaggccgactacgagaagcacaaggtgtacgcctgcgaggtgacccaccagggcctgagcagccccgtgaccaagagcttcaaccgcggcgagtgc

SEQ ID NO: 39 - protein, 449 aa, Artificial Sequence
  erb-Fc9
QVQLKQSGPGLVQPSQSLSITCTVSGFSLTNYGVHWVRQSPGKGLEWLGVIWSGGNTDYNTPFTSRLSINKDNSKSQVFFKMNSLQSNDTAIYYCARALTYYDYEFAYWGQGTLVTVSAASTKGPSVFPLAPSSKSTSGGTAALGCLVKDYFPEPVTVSWNSGALTSGVHTFPAVLQSSGLYSLSSVVTVPSSSLGTQTYICNVNHKPSNTKVDKRVEPKSCDKTHTCPPCPAPELLGGPSVFLFPPKPKDTLMISRTPEVTCVVVDVSHEDPEVKFNWYVDGVEVHNAKTKPREEQYNSTYRVVSVLTVLHQDWLNGKEYKCKVSNKALPAPIEKTISKAKGQPREPQVYTLPPSRDELTKNQVSLWCLVKGFYPSDIAVEWESNGQPENNYKTTPPVLDSDGSFFLYSALTVDKSRWQQGNVFSCSVMHEALHNHYTQKSLSLSPGK

SEQ ID NO: 40 - DNA, 1347 bp, Artificial Sequence
  nucleic acid molecules encoding erb-Fc9
caggtgcagctgaagcagagcggccccggcctggtgcagcccagccagagcctgagcatcacctgcaccgtgagcggcttcagcctgaccaactacggcgtgcactgggtgcgccagagccccggcaagggcctggagtggctgggcgtgatctggagcggcggcaacaccgactacaacacccccttcaccagccgcctgagcatcaacaaggacaacagcaagagccaggtgttcttcaagatgaacagcctgcagagcaacgacaccgccatctactactgcgcccgcgccctgacctactacgactacgagttcgcctactggggccagggcaccctggtgaccgtgagcgccgccagcactaaggggccctctgtgtttccactcgccccttctagcaaaagcacttccggaggaactgccgctctgggctgtctggtgaaagattacttccccgaaccagtcactgtgtcatggaactctggagcactgacatctggagttcacacctttcctgctgtgctgcagagttctggactgtactccctgtcatctgtggtcaccgtgccatcttcatctctggggacccagacctacatctgtaacgtgaaccacaaaccctccaacacaaaagtggacaaacgagtcgaaccaaaatcttgtgacaaaacccacacatgcccaccgtgcccagctccggaactcctgggcggaccgtcagtcttcctcttccccccaaaacccaaggacaccctcatgatctcccggacccctgaggtcacatgcgtggtggtggacgtgagccacgaagaccctgaggtcaagttcaactggtacgtggacggcgtggaggtgcataatgccaagacaaagccgcgggaggagcagtacaacagcacgtaccgtgtggtcagcgtcctcaccgtcctgcaccaggactggctgaatggcaaggagtacaagtgcaaggtctccaacaaagccctcccagcccccatcgagaaaaccatctccaaagccaaagggcagccccgagaaccacaggtgtacaccctgcccccaagtcgggatgagctgaccaagaaccaggtcagcctgtggtgcctggtcaaaggcttctatcccagcgacatcgccgtggagtgggagagcaatgggcagccggagaacaactacaagaccacgcctcccgtgttggactccgacggctccttcttcctctacagcgcgctcaccgtggacaagagcaggtggcagcaggggaacgtcttctcatgctccgtgatgcatgaggctctgcacaaccactacacgcagaagagcctctccctgtctccgggtaaa

SEQ ID NO: 41 - protein, 346 aa, Artificial Sequence
  Erb-Fc6
QVQLKQSGPGLVQPSQSLSITCTVSGFSLTNYGVHWVRQSPGKGLEWLGVIWSGGNTDYNTPFTSRLSINKDNSKSQVFFKMNSLQSNDTAIYYCARALTYYDYEFAYWGQGTLVTVSADKTHTCPPCPAPELLGGPSVFLFPPKPKDTLMISRTPEVTCVVVDVSHEDPEVKFNWYVDGVEVHNAKTKPREEQYNSTYRVVSVLTVLHQDWLNGKEYKCKVSNKALPAPIEKTISKAKGQPREPQVYTLPPSRDELTKNQVSLSCGVKGFYPSDIAVEWESNGQPENNYKTTPPVLDSDGSFKLASKLTVDKSRWQQGNVFSCSVMHEALHNHYTQKSLSLSPGK

SEQ ID NO: 42 - DNA, 1038 bp, Artificial Sequence
  nucleic acid molecules encoding Erb-Fc6
caggtgcagctgaagcagagcggccccggcctggtgcagcccagccagagcctgagcatcacctgcaccgtgagcggcttcagcctgaccaactacggcgtgcactgggtgcgccagagccccggcaagggcctggagtggctgggcgtgatctggagcggcggcaacaccgactacaacacccccttcaccagccgcctgagcatcaacaaggacaacagcaagagccaggtgttcttcaagatgaacagcctgcagagcaacgacaccgccatctactactgcgcccgcgccctgacctactacgactacgagttcgcctactggggccagggcaccctggtgaccgtgagcgccgacaagacccacacttgccccccttgtcccgctccggaactcctgggcggaccgtcagtcttcctcttccccccaaaacccaaggacaccctcatgatctcccggacccctgaggtcacatgcgtggtggtggacgtgagccacgaagaccctgaggtcaagttcaactggtacgtggacggcgtggaggtgcataatgccaagacaaagccgcgggaggagcagtacaacagcacgtaccgtgtggtcagcgtcctcaccgtcctgcaccaggactggctgaatggcaaggagtacaagtgcaaggtctccaacaaagccctcccagcccccatcgagaaaaccatctccaaagccaaagggcagccccgagaaccacaggtgtataccctgcccccatcccgggatgagctgaccaagaaccaggtcagcctgagttgcggggtcaaaggcttctatcccagcgacatcgccgtggagtgggagagcaatgggcagccggagaacaactacaagaccacgcctcccgtgttggactccgacggctccttcaagctcgccagcaagctcaccgtggacaagagcaggtggcagcaggggaacgtcttctcatgctccgtgatgcatgaggctctgcacaaccactacacgcagaagagcctctccctgtctccgggtaaa

SEQ ID NO: 43 - protein, 449 aa, Artificial Sequence
  Erb-Knob
QVQLKQSGPGLVQPSQSLSITCTVSGFSLTNYGVHWVRQSPGKGLEWLGVIWSGGNTDYNTPFTSRLSINKDNSKSQVFFKMNSLQSNDTAIYYCARALTYYDYEFAYWGQGTLVTVSAASTKGPSVFPLAPSSKSTSGGTAALGCLVKDYFPEPVTVSWNSGALTSGVHTFPAVLQSSGLYSLSSVVTVPSSSLGTQTYICNVNHKPSNTKVDKRVEPKSCDKTHTCPPCPAPELLGGPSVFLFPPKPKDTLMISRTPEVTCVVVDVSHEDPEVKFNWYVDGVEVHNAKTKPREEQYNSTYRVVSVLTVLHQDWLNGKEYKCKVSNKALPAPIEKTISKAKGQPREPQVYTLPPCRDELTKNQVSLWCLVKGFYPSDIAVEWESNGQPENNYKTTPPVLDSDGSFFLYSKLTVDKSRWQQGNVFSCSVMHEALHNHYTQKSLSLSPGK

SEQ ID NO: 44 - DNA, 1347 bp, Artificial Sequence
  nucleic acid molecules encoding Erb-Knob
caggtgcagctgaagcagagcggccccggcctggtgcagcccagccagagcctgagcatcacctgcaccgtgagcggcttcagcctgaccaactacggcgtgcactgggtgcgccagagccccggcaagggcctggagtggctgggcgtgatctggagcggcggcaacaccgactacaacacccccttcaccagccgcctgagcatcaacaaggacaacagcaagagccaggtgttcttcaagatgaacagcctgcagagcaacgacaccgccatctactactgcgcccgcgccctgacctactacgactacgagttcgcctactggggccagggcaccctggtgaccgtgagcgccgccagcaccaagggccccagcgtgttccccctggcccccagcagcaagagcaccagcggcggcaccgccgccctgggctgcctggtgaaggactacttccccgagcccgtgaccgtgagctggaacagcggcgccctgaccagcggcgtgcacaccttccccgccgtgctgcagagcagcggcctgtacagcctgagcagcgtggtgaccgtgcccagcagcagcctgggcacccagacctacatctgcaacgtgaaccacaagcccagcaacaccaaggtggacaagcgcgtggagcccaagagctgcgacaagacccacacctgccccccctgccccgcccccgagctgctgggcggccccagcgtgttcctgttcccccccaagcccaaggacaccctgatgatcagccgcacccccgaggtgacctgcgtggtggtggacgtgagccacgaggaccccgaggtgaagttcaactggtacgtggacggcgtggaggtgcacaacgccaagaccaagccccgcgaggagcagtacaacagcacctaccgcgtggtgagcgtgctgaccgtgctgcaccaggactggctgaacggcaaggagtacaagtgcaaggtgagcaacaaggccctgcccgcccccatcgagaagaccatcagcaaggccaagggccagccccgcgagccccaggtgtacaccctgcccccctgccgcgacgagctgaccaagaaccaggtgagcctgtggtgcctggtgaagggcttctaccccagcgacatcgccgtggagtgggagagcaacggccagcccgagaacaactacaagaccaccccccccgtgctggacagcgacggcagcttcttcctgtacagcaagctgaccgtggacaagagccgctggcagcagggcaacgtgttcagctgcagcgtgatgcacgaggccctgcacaaccactacacccagaagagcctgagcctgagccccggcaag

SEQ ID NO: 45 - protein, 214 aa, Artificial Sequence
  T-LC
DIQMTQSPSSLSASVGDRVTITCRASQDVNTAVAWYQQKPGKAPKLLIYSASFLYSGVPSRFSGSRSGTDFTLTISSLQPEDFATYYCQQHYTTPPTFGQGTKVEIKRTVAAPSVFIFPPSDEQLKSGTASVVCLLNNFYPREAKVQWKVDNALQSGNSQESVTEQDSKDSTYSLSSTLTLSKADYEKHKVYACEVTHQGLSSPVTKSFNRGEC

SEQ ID NO: 46 - DNA, 708 bp, Artificial Sequence
  nucleic acid molecules encoding T-LC
gacatccagatgacccagagccccagcagcctgagcgccagcgtgggcgaccgcgtgaccatcacctgccgcgccagccaggacgtgaacaccgccgtggcctggtaccagcagaagcccggcaaggcccccaagctgctgatctacagcgccagcttcctgtacagcggcgtgcccagccgcttcagcggcagccgcagcggcaccgacttcaccctgaccatcagcagcctgcagcccgaggacttcgccacctactactgccagcagcactacaccaccccccccaccttcggccagggcaccaaggtggagatcaaatactactgccagcagaacaacaactggcccaccaccttcggcgccggcaccaagctggagctgaagcgcaccgtggccgcccccagcgtgttcatcttcccccccagcgacgagcagctgaagagcggcaccgccagcgtggtgtgcctgctgaacaacttctacccccgcgaggccaaggtgcagtggaaggtggacaacgccctgcagagcggcaacagccaggagagcgtgaccgagcaggacagcaaggacagcacctacagcctgagcagcaccctgaccctgagcaaggccgactacgagaagcacaaggtgtacgcctgcgaggtgacccaccagggcctgagcagccccgtgaccaagagcttcaaccgcggcgagtgc

SEQ ID NO: 47 - protein, 450 aa, Artificial Sequence
  T-Fc9
EVQLVESGGGLVQPGGSLRLSCAASGFNIKDTYIHWVRQAPGKGLEWVARIYPTNGYTRYADSVKGRFTISADTSKNTAYLQMNSLRAEDTAVYYCSRWGGDGFYAMDYWGQGTLVTVSSASTKGPSVFPLAPSSKSTSGGTAALGCLVKDYFPEPVTVSWNSGALTSGVHTFPAVLQSSGLYSLSSVVTVPSSSLGTQTYICNVNHKPSNTKVDKRVEPKSCDKTHTCPPCPAPELLGGPSVFLFPPKPKDTLMISRTPEVTCVVVDVSHEDPEVKFNWYVDGVEVHNAKTKPREEQYNSTYRVVSVLTVLHQDWLNGKEYKCKVSNKALPAPIEKTISKAKGQPREPQVYTLPPSRDELTKNQVSLWCLVKGFYPSDIAVEWESNGQPENNYKTTPPVLDSDGSFFLYSALTVDKSRWQQGNVFSCSVMHEALHNHYTQKSLSLSPGK

SEQ ID NO: 48 - DNA, 1350 bp, Artificial Sequence
  nucleic acid molecules encoding T-Fc9
gaggtgcagctggtggagagcggcggcggcctggtgcagcccggcggcagcctgcgcctgagctgcgccgccagcggcttcaacatcaaggacacctacatccactgggtgcgccaggcccccggcaagggcctggagtgggtggcccgcatctaccccaccaacggctacacccgctacgccgacagcgtgaagggccgcttcaccatcagcgccgacaccagcaagaacaccgcctacctgcagatgaacagcctgcgcgccgaggacaccgccgtgtactactgcagccgctggggcggcgacggcttctacgccatggactactggggccagggcaccctggtgaccgtgagcagcgccagcactaaggggccctctgtgtttccactcgccccttctagcaaaagcacttccggaggaactgccgctctgggctgtctggtgaaagattacttccccgaaccagtcactgtgtcatggaactctggagcactgacatctggagttcacacctttcctgctgtgctgcagagttctggactgtactccctgtcatctgtggtcaccgtgccatcttcatctctggggacccagacctacatctgtaacgtgaaccacaaaccctccaacacaaaagtggacaaacgagtcgaaccaaaatcttgtgacaaaacccacacatgcccaccgtgcccagctccggaactcctgggcggaccgtcagtcttcctcttccccccaaaacccaaggacaccctcatgatctcccggacccctgaggtcacatgcgtggtggtggacgtgagccacgaagaccctgaggtcaagttcaactggtacgtggacggcgtggaggtgcataatgccaagacaaagccgcgggaggagcagtacaacagcacgtaccgtgtggtcagcgtcctcaccgtcctgcaccaggactggctgaatggcaaggagtacaagtgcaaggtctccaacaaagccctcccagcccccatcgagaaaaccatctccaaagccaaagggcagccccgagaaccacaggtgtacaccctgcccccaagtcgggatgagctgaccaagaaccaggtcagcctgtggtgcctggtcaaaggcttctatcccagcgacatcgccgtggagtgggagagcaatgggcagccggagaacaactacaagaccacgcctcccgtgttggactccgacggctccttcttcctctacagcgcgctcaccgtggacaagagcaggtggcagcaggggaacgtcttctcatgctccgtgatgcatgaggctctgcacaaccactacacgcagaagagcctctccctgtctccgggtaaa

SEQ ID NO: 49 - protein, 214 aa, Artificial Sequence
  P-LC
DIQMTQSPSSLSASVGDRVTITCKASQDVSIGVAWYQQKPGKAPKLLIYSASYRYTGVPSRFSGSGSGTDFTLTISSLQPEDFATYYCQQYYIYPYTFGQGTKVEIKRTVAAPSVFIFPPSDEQLKSGTASVVCLLNNFYPREAKVQWKVDNALQSGNSQESVTEQDSKDSTYSLSSTLTLSKADYEKHKVYACEVTHQGLSSPVTKSFNRGEC

SEQ ID NO: 50 - DNA, 708 bp, Artificial Sequence
  nucleic acid molecules encoding P-LC
gacatccagatgacccagagccccagcagcctgagcgccagcgtgggcgaccgcgtgaccatcacctgcaaggccagccaggacgtgagcatcggcgtggcctggtaccagcagaagcccggcaaggcccccaagctgctgatctacagcgccagctaccgctacaccggcgtgcccagccgcttcagcggcagcggcagcggcaccgacttcaccctgaccatcagcagcctgcagcccgaggacttcgccacctactactgccagcagtactacatctacccctacaccttcggccagggcaccaaggtggagatcaagtactactgccagcagaacaacaactggcccaccaccttcggcgccggcaccaagctggagctgaagcgcaccgtggccgcccccagcgtgttcatcttcccccccagcgacgagcagctgaagagcggcaccgccagcgtggtgtgcctgctgaacaacttctacccccgcgaggccaaggtgcagtggaaggtggacaacgccctgcagagcggcaacagccaggagagcgtgaccgagcaggacagcaaggacagcacctacagcctgagcagcaccctgaccctgagcaaggccgactacgagaagcacaaggtgtacgcctgcgaggtgacccaccagggcctgagcagccccgtgaccaagagcttcaaccgcggcgagtgc

SEQ ID NO: 51 - protein, 449 aa, Artificial Sequence
  P-Fc9
EVQLVESGGGLVQPGGSLRLSCAASGFTFTDYTMDWVRQAPGKGLEWVADVNPNSGGSIYNQRFKGRFTLSVDRSKNTLYLQMNSLRAEDTAVYYCARNLGPSFYFDYWGQGTLVTVSSASTKGPSVFPLAPSSKSTSGGTAALGCLVKDYFPEPVTVSWNSGALTSGVHTFPAVLQSSGLYSLSSVVTVPSSSLGTQTYICNVNHKPSNTKVDKRVEPKSCDKTHTCPPCPAPELLGGPSVFLFPPKPKDTLMISRTPEVTCVVVDVSHEDPEVKFNWYVDGVEVHNAKTKPREEQYNSTYRVVSVLTVLHQDWLNGKEYKCKVSNKALPAPIEKTISKAKGQPREPQVYTLPPSRDELTKNQVSLWCLVKGFYPSDIAVEWESNGQPENNYKTTPPVLDSDGSFFLYSALTVDKSRWQQGNVFSCSVMHEALHNHYTQKSLSLSPGK

SEQ ID NO: 52 - DNA, 1347 bp, Artificial Sequence
  nucleic acid molecules encoding P-Fc9
gaggtgcagctggtggagagcggcggcggcctggtgcagcccggcggcagcctgcgcctgagctgcgccgccagcggcttcaccttcaccgactacaccatggactgggtgcgccaggcccccggcaagggcctggagtgggtggccgacgtgaaccccaacagcggcggcagcatctacaaccagcgcttcaagggccgcttcaccctgagcgtggaccgcagcaagaacaccctgtacctgcagatgaacagcctgcgcgccgaggacaccgccgtgtactactgcgcccgcaacctgggccccagcttctacttcgactactggggccagggcaccctggtgaccgtgagcagcgccagcactaaggggccctctgtgtttccactcgccccttctagcaaaagcacttccggaggaactgccgctctgggctgtctggtgaaagattacttccccgaaccagtcactgtgtcatggaactctggagcactgacatctggagttcacacctttcctgctgtgctgcagagttctggactgtactccctgtcatctgtggtcaccgtgccatcttcatctctggggacccagacctacatctgtaacgtgaaccacaaaccctccaacacaaaagtggacaaacgagtcgaaccaaaatcttgtgacaaaacccacacatgcccaccgtgcccagctccggaactcctgggcggaccgtcagtcttcctcttccccccaaaacccaaggacaccctcatgatctcccggacccctgaggtcacatgcgtggtggtggacgtgagccacgaagaccctgaggtcaagttcaactggtacgtggacggcgtggaggtgcataatgccaagacaaagccgcgggaggagcagtacaacagcacgtaccgtgtggtcagcgtcctcaccgtcctgcaccaggactggctgaatggcaaggagtacaagtgcaaggtctccaacaaagccctcccagcccccatcgagaaaaccatctccaaagccaaagggcagccccgagaaccacaggtgtacaccctgcccccaagtcgggatgagctgaccaagaaccaggtcagcctgtggtgcctggtcaaaggcttctatcccagcgacatcgccgtggagtgggagagcaatgggcagccggagaacaactacaagaccacgcctcccgtgttggactccgacggctccttcttcctctacagcgcgctcaccgtggacaagagcaggtggcagcaggggaacgtcttctcatgctccgtgatgcatgaggctctgcacaaccactacacgcagaagagcctctccctgtctccgggtaaa

SEQ ID NO: 53 - protein, 214 aa, Artificial Sequence
  Mab806-LC
DILMTQSPSSMSVSLGDTVSITCHSSQDINSNIGWLQQRPGKSFKGLIYHGTNLDDEVPSRFSGSGSGADYSLTISSLESEDFADYYCVQYAQFPWTFGGGTKLEIKRTVAAPSVFIFPPSDEQLKSGTASVVCLLNNFYPREAKVQWKVDNALQSGNSQESVTEQDSKDSTYSLSSTLTLSKADYEKHKVYACEVTHQGLSSPVTKSFNRGEC

SEQ ID NO: 54 - DNA, 708 bp, Artificial Sequence
  nucleic acid molecules encoding Mab806-LC
gacatcctgatgacccagagccccagcagcatgagcgtgagcctgggcgacaccgtgagcatcacctgccacagcagccaggacatcaacagcaacatcggctggctgcagcagcgccccggcaagagcttcaagggcctgatctaccacggcaccaacctggacgacgaggtgcccagccgcttcagcggcagcggcagcggcgccgactacagcctgaccatcagcagcctggagagcgaggacttcgccgactactactgcgtgcagtacgcccagttcccctggaccttcggcggcggcaccaagctggagatcaagtactactgccagcagaacaacaactggcccaccaccttcggcgccggcaccaagctggagctgaagcgcaccgtggccgcccccagcgtgttcatcttcccccccagcgacgagcagctgaagagcggcaccgccagcgtggtgtgcctgctgaacaacttctacccccgcgaggccaaggtgcagtggaaggtggacaacgccctgcagagcggcaacagccaggagagcgtgaccgagcaggacagcaaggacagcacctacagcctgagcagcaccctgaccctgagcaaggccgactacgagaagcacaaggtgtacgcctgcgaggtgacccaccagggcctgagcagccccgtgaccaagagcttcaaccgcggcgagtgc

SEQ ID NO: 55 - protein, 446 aa, Artificial Sequence
  Mab806-Fc9
DVQLQESGPSLVKPSQSLSLTCTVTGYSITSDFAWNWIRQFPGNKLEWMGYISYSGNTRYNPSLKSRISITRDTSKNQFFLQLNSVTIEDTATYYCVTAGRGFPYWGQGTLVTVSAASTKGPSVFPLAPSSKSTSGGTAALGCLVKDYFPEPVTVSWNSGALTSGVHTFPAVLQSSGLYSLSSVVTVPSSSLGTQTYICNVNHKPSNTKVDKRVEPKSCDKTHTCPPCPAPELLGGPSVFLFPPKPKDTLMISRTPEVTCVVVDVSHEDPEVKFNWYVDGVEVHNAKTKPREEQYNSTYRVVSVLTVLHQDWLNGKEYKCKVSNKALPAPIEKTISKAKGQPREPQVYTLPPSRDELTKNQVSLWCLVKGFYPSDIAVEWESNGQPENNYKTTPPVLDSDGSFFLYSALTVDKSRWQQGNVFSCSVMHEALHNHYTQKSLSLSPGK

SEQ ID NO: 56 - DNA, 1338 bp, Artificial Sequence
  nucleic acid molecules encoding Mab806-Fc9
gacgtgcagctgcaggagagcggccccagcctggtgaagcccagccagagcctgagcctgacctgcaccgtgaccggctacagcatcaccagcgacttcgcctggaactggatccgccagttccccggcaacaagctggagtggatgggctacatcagctacagcggcaacacccgctacaaccccagcctgaagagccgcatcagcatcacccgcgacaccagcaagaaccagttcttcctgcagctgaacagcgtgaccatcgaggacaccgccacctactactgcgtgaccgccggccgcggcttcccctactggggccagggcaccctggtgaccgtgagcgccgccagcactaaggggccctctgtgtttccactcgccccttctagcaaaagcacttccggaggaactgccgctctgggctgtctggtgaaagattacttccccgaaccagtcactgtgtcatggaactctggagcactgacatctggagttcacacctttcctgctgtgctgcagagttctggactgtactccctgtcatctgtggtcaccgtgccatcttcatctctggggacccagacctacatctgtaacgtgaaccacaaaccctccaacacaaaagtggacaaacgagtcgaaccaaaatcttgtgacaaaacccacacatgcccaccgtgcccagctccggaactcctgggcggaccgtcagtcttcctcttccccccaaaacccaaggacaccctcatgatctcccggacccctgaggtcacatgcgtggtggtggacgtgagccacgaagaccctgaggtcaagttcaactggtacgtggacggcgtggaggtgcataatgccaagacaaagccgcgggaggagcagtacaacagcacgtaccgtgtggtcagcgtcctcaccgtcctgcaccaggactggctgaatggcaaggagtacaagtgcaaggtctccaacaaagccctcccagcccccatcgagaaaaccatctccaaagccaaagggcagccccgagaaccacaggtgtacaccctgcccccaagtcgggatgagctgaccaagaaccaggtcagcctgtggtgcctggtcaaaggcttctatcccagcgacatcgccgtggagtgggagagcaatgggcagccggagaacaactacaagaccacgcctcccgtgttggactccgacggctccttcttcctctacagcgcgctcaccgtggacaagagcaggtggcagcaggggaacgtcttctcatgctccgtgatgcatgaggctctgcacaaccactacacgcagaagagcctctccctgtctccgggtaaa

SEQ ID NO: 57 - protein, 219 aa, Artificial Sequence
  C-MAB-LC
DVVMTQSPLSLPVTPGEPASISCRSSQSLVHSNRNTYLHWYLQKPGQSPQLLIYKVSNRFSGVPDRFSGSGSGTDFTLKISRVEAEDVGVYYCSQNTHVPPTFGQGTKLEIKRTVAAPSVFIFPPSDEQLKSGTASVVCLLNNFYPREAKVQWKVDNALQSGNSQESVTEQDSKDSTYSLSSTLTLSKADYEKHKVYACEVTHQGLSSPVTKSFNRGEC

SEQ ID NO: 58 - DNA, 657 bp, Artificial Sequence
  nucleic acid molecules encoding C-MAB-LC
gacgtggtgatgacccagagccccctgagcctgcctgtgacacctggcgagcctgccagcatcagctgcagaagcagccagtccctggtgcacagcaacaggaacacctacctgcactggtatttacagaagcccggacagagcccccagctgctgatctacaaggtgagcaacaggttcagcggcgtgcctgacaggttttccggcagcggcagcggcaccgacttcaccctgaagatcagcagggtggaggccgaggatgtgggcgtgtactactgcagccagaacacccacgtgccccctacctttggccagggcaccaagctggagatcaagcgtacggtggctgcaccatctgtcttcatcttcccgccatctgatgagcagttgaaatctggtaccgctagcgttgtgtgcctgctgaataacttttatccacgggaggctaaggtgcagtggaaagtggacaatgccctccagagcggaaatagccaagagtccgttaccgaacaggactctaaagactctacatactccctgtcctccacactgaccctctccaaggccgactatgagaaacacaaggtttacgcatgcgaggtcacacaccagggactctcctctcccgtgaccaagagcttcaaccggggagaatgc

SEQ ID NO: 59 - protein, 445 aa, Artificial Sequence
  C-MAB-Fc9
QVQLVQSGAEVKKPGASVKVSCKASGYTFTDYEMHWVRQAPGQGLEWMGALDPKTGDTAYSQKFKGRVTLTADKSTSTAYMELSSLTSEDTAVYYCTRFYSYTYWGQGTLVTVSSASTKGPSVFPLAPSSKSTSGGTAALGCLVKDYFPEPVTVSWNSGALTSGVHTFPAVLQSSGLYSLSSVVTVPSSSLGTQTYICNVNHKPSNTKVDKRVEPKSCDKTHTCPPCPAPELLGGPSVFLFPPKPKDTLMISRTPEVTCVVVDVSHEDPEVKFNWYVDGVEVHNAKTKPREEQYNSTYRVVSVLTVLHQDWLNGKEYKCKVSNKALPAPIEKTISKAKGQPREPQVYTLPPSRDELTKNQVSLWCLVKGFYPSDIAVEWESNGQPENNYKTTPPVLDSDGSFFLYSALTVDKSRWQQGNVFSCSVMHEALHNHYTQKSLSLSPGK

SEQ ID NO: 60 - DNA, 1335 bp, Artificial Sequence
  nucleic acid molecules encoding C-MAB-Fc9
caggtgcagctggtgcagagcggcgccgaggtgaagaaacctggcgccagcgtgaaggtgagctgcaaggcctccggctacaccttcaccgactacgagatgcactgggtgaggcaggcccctggacaaggactggagtggatgggcgccttagatcctaagacaggcgacaccgcctactcccagaagttcaagggcagggtgaccctgaccgccgacaagagcaccagcaccgcctacatggagctgagcagcctgaccagcgaggacaccgccgtgtactattgcaccaggttctacagctacacctactggggccagggcacactggtgaccgtgagcagcgccagcactaaggggccctctgtgtttccactcgccccttctagcaaaagcacttccggaggaactgccgctctgggctgtctggtgaaagattacttccccgaaccagtcactgtgtcatggaactctggagcactgacatctggagttcacacctttcctgctgtgctgcagagttctggactgtactccctgtcatctgtggtcaccgtgccatcttcatctctggggacccagacctacatctgtaacgtgaaccacaaaccctccaacacaaaagtggacaaacgagtcgaaccaaaatcttgtgacaaaacccacacatgcccaccgtgcccagctccggaactcctgggcggaccgtcagtcttcctcttccccccaaaacccaaggacaccctcatgatctcccggacccctgaggtcacatgcgtggtggtggacgtgagccacgaagaccctgaggtcaagttcaactggtacgtggacggcgtggaggtgcataatgccaagacaaagccgcgggaggagcagtacaacagcacgtaccgtgtggtcagcgtcctcaccgtcctgcaccaggactggctgaatggcaaggagtacaagtgcaaggtctccaacaaagccctcccagcccccatcgagaaaaccatctccaaagccaaagggcagccccgagaaccacaggtgtacaccctgcccccaagtcgggatgagctgaccaagaaccaggtcagcctgtggtgcctggtcaaaggcttctatcccagcgacatcgccgtggagtgggagagcaatgggcagccggagaacaactacaagaccacgcctcccgtgttggactccgacggctccttcttcctctacagcgcgctcaccgtggacaagagcaggtggcagcaggggaacgtcttctcatgctccgtgatgcatgaggctctgcacaaccactacacgcagaagagcctctccctgtctccgggtaaa

SEQ ID NO: 61 - protein, 215 aa, Artificial Sequence
  28H1-LC
EIVLTQSPGTLSLSPGERATLSCRASQSVSRSYLAWYQQKPGQAPRLLIIGASTRATGIPDRFSGSGSGTDFTLTISRLEPEDFAVYYCQQGQVIPPTFGQGTKVEIKRTVAAPSVFIFPPSDEQLKSGTASVVCLLNNFYPREAKVQWKVDNALQSGNSQESVTEQDSKDSTYSLSSTLTLSKADYEKHKVYACEVTHQGLSSPVTKSFNRGEC

SEQ ID NO: 62 - DNA, 645 bp, Artificial Sequence
  nucleic acid molecules encoding 28H1-LC
gagatcgtgctgacacagtctccaggcaccctgtctctgtctccaggagagagagccaccctgtcttgcagagcctctcagagcgtgtccaggagctacctggcttggtatcagcagaagccaggacaggcccctagactgctgatcatcggagcctctacaagagccacaggcatcccagacagattcagcggcagcggaagcggcacagacttcaccctgaccatcagcaggctggagccagaggacttcgccgtgtactattgccagcagggccaggtcatccctcctacctttggacagggcaccaaggtggagatcaagcgtacggtggctgcaccatctgtcttcatcttcccgccatctgatgagcagttgaaatctggtaccgctagcgttgtgtgcctgctgaataacttttatccacgggaggctaaggtgcagtggaaagtggacaatgccctccagagcggaaatagccaagagtccgttaccgaacaggactctaaagactctacatactccctgtcctccacactgaccctctccaaggccgactatgagaaacacaaggtttacgcatgcgaggtcacacaccagggactctcctctcccgtgaccaagagcttcaaccggggagaatgc

SEQ ID NO: 63 - protein, 446 aa, Artificial Sequence
  28H1-Fc9
EVQLLESGGGLVQPGGSLRLSCAASGFTFSSHAMSWVRQAPGKGLEWVSAIWASGEQYYADSVKGRFTISRDNSKNTLYLQMNSLRAQDTAVYYCAKGWLGNFDYWGQGTLVTVSSASTKGPSVFPLAPSSKSTSGGTAALGCLVKDYFPEPVTVSWNSGALTSGVHTFPAVLQSSGLYSLSSVVTVPSSSLGTQTYICNVNHKPSNTKVDKRVEPKSCDKTHTCPPCPAPELLGGPSVFLFPPKPKDTLMISRTPEVTCVVVDVSHEDPEVKFNWYVDGVEVHNAKTKPREEQYNSTYRVVSVLTVLHQDWLNGKEYKCKVSNKALPAPIEKTISKAKGQPREPQVYTLPPSRDELTKNQVSLWCLVKGFYPSDIAVEWESNGQPENNYKTTPPVLDSDGSFFLYSALTVDKSRWQQGNVFSCSVMHEALHNHYTQKSLSLSPGK

SEQ ID NO: 64 - DNA, 1338 bp, Artificial Sequence
  nucleic acid molecules encoding 28H1-Fc9
gaggtgcagctgctggaatcaggaggaggactggtgcagccaggaggatctctgagactgtcttgcgccgccagcggctttacattcagctctcacgccatgtcttgggtccgacaggctccaggcaaaggactggaatgggtgtccgctatttgggccagcggagagcagtactacgccgacagcgtgaagggacggttcaccatcagccgggacaacagcaagaacaccctgtacctgcagatgaacagcctgagggcccaggataccgccgtgtactattgcgccaagggttggctgggcaacttcgactattggggccagggaaccctggtgacagtgtccagcgccagcactaaggggccctctgtgtttccactcgccccttctagcaaaagcacttccggaggaactgccgctctgggctgtctggtgaaagattacttccccgaaccagtcactgtgtcatggaactctggagcactgacatctggagttcacacctttcctgctgtgctgcagagttctggactgtactccctgtcatctgtggtcaccgtgccatcttcatctctggggacccagacctacatctgtaacgtgaaccacaaaccctccaacacaaaagtggacaaacgagtcgaaccaaaatcttgtgacaaaacccacacatgcccaccgtgcccagctccggaactcctgggcggaccgtcagtcttcctcttccccccaaaacccaaggacaccctcatgatctcccggacccctgaggtcacatgcgtggtggtggacgtgagccacgaagaccctgaggtcaagttcaactggtacgtggacggcgtggaggtgcataatgccaagacaaagccgcgggaggagcagtacaacagcacgtaccgtgtggtcagcgtcctcaccgtcctgcaccaggactggctgaatggcaaggagtacaagtgcaaggtctccaacaaagccctcccagcccccatcgagaaaaccatctccaaagccaaagggcagccccgagaaccacaggtgtacaccctgcccccaagtcgggatgagctgaccaagaaccaggtcagcctgtggtgcctggtcaaaggcttctatcccagcgacatcgccgtggagtgggagagcaatgggcagccggagaacaactacaagaccacgcctcccgtgttggactccgacggctccttcttcctctacagcgcgctcaccgtggacaagagcaggtggcagcaggggaacgtcttctcatgctccgtgatgcatgaggctctgcacaaccactacacgcagaagagcctctccctgtctccgggtaaa

SEQ ID NO: 65 - protein, 220 aa, Artificial Sequence
  5E5-LC
ELVMTQSPSSLTVTAGEKVTMICKSSQSLLNSGDQKNYLTWYQQKPGQPPKLLIFWASTRESGVPDRFTGSGSGTDFTLTISSVQAEDLAVYYCQNDYSYPLTFGAGTKLELKRTVAAPSVFIFPPSDEQLKSGTASVVCLLNNFYPREAKVQWKVDNALQSGNSQESVTEQDSKDSTYSLSSTLTLSKADYEKHKVYACEVTHQGLSSPVTKSFNRGEC

SEQ ID NO: 66 - DNA, 660 bp, Artificial Sequence
  nucleic acid molecules encoding 5E5-LC
gaactcgtgatgacccagagccccagctctctgacagtgacagccggcgagaaagtgaccatgatctgcaagtcctcccagagcctgctgaactccggcgaccagaagaactacctgacctggtatcagcagaaacccggccagccccccaagctgctgatcttttgggccagcacccgggaaagcggcgtgcccgatagattcacaggcagcggctccggcaccgactttaccctgaccatcagctccgtgcaggccgaggacctggccgtgtattactgccagaacgactacagctaccccctgaccttcggagccggcaccaagctggaactgaagcgtacggtggctgcaccatctgtcttcatcttcccgccatctgatgagcagttgaaatctggtaccgctagcgttgtgtgcctgctgaataacttttatccacgggaggctaaggtgcagtggaaagtggacaatgccctccagagcggaaatagccaagagtccgttaccgaacaggactctaaagactctacatactccctgtcctccacactgaccctctccaaggccgactatgagaaacacaaggtttacgcatgcgaggtcacacaccagggactctcctctcccgtgaccaagagcttcaaccggggagaatgc

SEQ ID NO: 67 - protein, 446 aa, Artificial Sequence
  5E5-Fc9
QVQLQQSDAELVKPGSSVKISCKASGYTFTDHAIHWVKQKPEQGLEWIGHFSPGNTDIKYNDKFKGKATLTVDRSSSTAYMQLNSLTSEDSAVYFCKTSTFFFDYWGQGTTLTVSSASTKGPSVFPLAPSSKSTSGGTAALGCLVKDYFPEPVTVSWNSGALTSGVHTFPAVLQSSGLYSLSSVVTVPSSSLGTQTYICNVNHKPSNTKVDKRVEPKSCDKTHTCPPCPAPELLGGPSVFLFPPKPKDTLMISRTPEVTCVVVDVSHEDPEVKFNWYVDGVEVHNAKTKPREEQYNSTYRVVSVLTVLHQDWLNGKEYKCKVSNKALPAPIEKTISKAKGQPREPQVYTLPPSRDELTKNQVSLWCLVKGFYPSDIAVEWESNGQPENNYKTTPPVLDSDGSFFLYSALTVDKSRWQQGNVFSCSVMHEALHNHYTQKSLSLSPGK

SEQ ID NO: 68 - DNA, 1338 bp, Artificial Sequence
  nucleic acid molecules encoding 5E5-Fc9
caggtgcagctgcagcagtctgatgccgagctcgtgaagcctggcagcagcgtgaagatcagctgcaaggccagcggctacaccttcaccgaccacgccatccactgggtcaagcagaagcctgagcagggcctggaatggatcggccacttcagccccggcaacaccgacatcaagtacaacgacaagttcaagggcaaggccaccctgaccgtggacagaagcagcagcaccgcctacatgcagctgaacagcctgaccagcgaggacagcgccgtgtacttctgcaagaccagcaccttctttttcgactactggggccagggcacaaccctgacagtgtctagcgccagcactaaggggccctctgtgtttccactcgccccttctagcaaaagcacttccggaggaactgccgctctgggctgtctggtgaaagattacttccccgaaccagtcactgtgtcatggaactctggagcactgacatctggagttcacacctttcctgctgtgctgcagagttctggactgtactccctgtcatctgtggtcaccgtgccatcttcatctctggggacccagacctacatctgtaacgtgaaccacaaaccctccaacacaaaagtggacaaacgagtcgaaccaaaatcttgtgacaaaacccacacatgcccaccgtgcccagctccggaactcctgggcggaccgtcagtcttcctcttccccccaaaacccaaggacaccctcatgatctcccggacccctgaggtcacatgcgtggtggtggacgtgagccacgaagaccctgaggtcaagttcaactggtacgtggacggcgtggaggtgcataatgccaagacaaagccgcgggaggagcagtacaacagcacgtaccgtgtggtcagcgtcctcaccgtcctgcaccaggactggctgaatggcaaggagtacaagtgcaaggtctccaacaaagccctcccagcccccatcgagaaaaccatctccaaagccaaagggcagccccgagaaccacaggtgtacaccctgcccccaagtcgggatgagctgaccaagaaccaggtcagcctgtggtgcctggtcaaaggcttctatcccagcgacatcgccgtggagtgggagagcaatgggcagccggagaacaactacaagaccacgcctcccgtgttggactccgacggctccttcttcctctacagcgcgctcaccgtggacaagagcaggtggcagcaggggaacgtcttctcatgctccgtgatgcatgaggctctgcacaaccactacacgcagaagagcctctccctgtctccgggtaaa

SEQ ID NO: 69 - protein, 213 aa, Artificial Sequence
  E-mab-LC
QVVLTQSPVIMSASPGEKVTMTCSASSSISYMYWYQQKPGTSPKRWIYDTSKLASGVPARFSGSGSGTSYSLTISNMEAGDAATYYCHQRDSYPWTFGGGTNLEIKRTVAAPSVFIFPPSDEQLKSGTASVVCLLNNFYPREAKVQWKVDNALQSGNSQESVTEQDSKDSTYSLSSTLTLSKADYEKHKVYACEVTHQGLSSPVTKSFNRGEC

SEQ ID NO: 70 - DNA, 639 bp, Artificial Sequence
  nucleic acid molecules encoding E-mab-LC
caggtggtgctgacccagagccccgtgatcatgtccgccagccctggcgagaaggtgaccatgacctgcagcgccagcagcagcatcagctacatgtactggtatcaacagaagcccggcaccagccccaagaggtggatctacgacaccagcaagctggctagcggcgtgcctgccagattcagcggaagcggcagcggcaccagctacagcctgaccatcagcaacatggaggccggcgacgccgccacatactactgccaccagagggactcctacccctggaccttcggcggaggcaccaacctggagatcaagcgtacggtggctgcaccatctgtcttcatcttcccgccatctgatgagcagttgaaatctggtaccgctagcgttgtgtgcctgctgaataacttttatccacgggaggctaaggtgcagtggaaagtggacaatgccctccagagcggaaatagccaagagtccgttaccgaacaggactctaaagactctacatactccctgtcctccacactgaccctctccaaggccgactatgagaaacacaaggtttacgcatgcgaggtcacacaccagggactctcctctcccgtgaccaagagcttcaaccggggagaatgc

SEQ ID NO: 71 - protein, 443 aa, Artificial Sequence
  E-mab-Fc9
QVQLKESGPDLVAPSQSLSITCTVSGFSLSKFGVNWVRQPPGKGLEWLGVIWGDGSTSYNSGLISRLSISKENSKSQVFLKLNSLQADDTATYYCVKPGGDYWGHGTSVTVSSASTKGPSVFPLAPSSKSTSGGTAALGCLVKDYFPEPVTVSWNSGALTSGVHTFPAVLQSSGLYSLSSVVTVPSSSLGTQTYICNVNHKPSNTKVDKRVEPKSCDKTHTCPPCPAPELLGGPSVFLFPPKPKDTLMISRTPEVTCVVVDVSHEDPEVKFNWYVDGVEVHNAKTKPREEQYNSTYRVVSVLTVLHQDWLNGKEYKCKVSNKALPAPIEKTISKAKGQPREPQVYTLPPSRDELTKNQVSLWCLVKGFYPSDIAVEWESNGQPENNYKTTPPVLDSDGSFFLYSALTVDKSRWQQGNVFSCSVMHEALHNHYTQKSLSLSPGK

SEQ ID NO: 72 - DNA, 1329 bp, Artificial Sequence
  nucleic acid molecules encoding E-mab-Fc9
caggtgcagctgaaggagagcggacctgacctggtggcccctagccagagcctgagcatcacctgcaccgtgagcggcttcagcctgagcaagttcggcgtgaactgggtgagacagccccccggaaagggactggagtggctgggagtgatctggggcgacggcagcaccagctacaacagcggcctgatcagcaggctgtccatcagcaaggagaacagcaagagccaggtgttcctgaagctgaacagcctgcaggccgacgacaccgccacctactactgcgtgaagcctggcggcgattactggggccacggaaccagcgtgaccgtgagcagcgccagcactaaggggccctctgtgtttccactcgccccttctagcaaaagcacttccggaggaactgccgctctgggctgtctggtgaaagattacttccccgaaccagtcactgtgtcatggaactctggagcactgacatctggagttcacacctttcctgctgtgctgcagagttctggactgtactccctgtcatctgtggtcaccgtgccatcttcatctctggggacccagacctacatctgtaacgtgaaccacaaaccctccaacacaaaagtggacaaacgagtcgaaccaaaatcttgtgacaaaacccacacatgcccaccgtgcccagctccggaactcctgggcggaccgtcagtcttcctcttccccccaaaacccaaggacaccctcatgatctcccggacccctgaggtcacatgcgtggtggtggacgtgagccacgaagaccctgaggtcaagttcaactggtacgtggacggcgtggaggtgcataatgccaagacaaagccgcgggaggagcagtacaacagcacgtaccgtgtggtcagcgtcctcaccgtcctgcaccaggactggctgaatggcaaggagtacaagtgcaaggtctccaacaaagccctcccagcccccatcgagaaaaccatctccaaagccaaagggcagccccgagaaccacaggtgtacaccctgcccccaagtcgggatgagctgaccaagaaccaggtcagcctgtggtgcctggtcaaaggcttctatcccagcgacatcgccgtggagtgggagagcaatgggcagccggagaacaactacaagaccacgcctcccgtgttggactccgacggctccttcttcctctacagcgcgctcaccgtggacaagagcaggtggcagcaggggaacgtcttctcatgctccgtgatgcatgaggctctgcacaaccactacacgcagaagagcctctccctgtctccgggtaaa

SEQ ID NO: 73 - protein, 213 aa, Artificial Sequence
  A-mab-LC
DIELTQSPAIMSASPGEKVTMTCSASSSVSYMHWYQQKSGTSPKRWIYDTSKLASGVPGRFSGSGSGNSYSLTISSVEAEDDATYYCQQWSKHPLTFGSGTKVEIKRTVAAPSVFIFPPSDEQLKSGTASVVCLLNNFYPREAKVQWKVDNALQSGNSQESVTEQDSKDSTYSLSSTLTLSKADYEKHKVYACEVTHQGLSSPVTKSFNRGEC

SEQ ID NO: 74 - DNA, 639 bp, Artificial Sequence
  nucleic acid molecules encoding A-mab-LC
gacatcgagctgacacagagccctgccatcatgtctgctagccctggcgagaaagtgaccatgacctgtagcgccagcagcagcgtgtcctacatgcactggtatcagcagaagtccggcacaagccccaagcggtggatctacgatacaagcaagctggcctctggcgtgcccggcagattttctggttctggcagcggcaacagctacagcctgacaatcagctccgtggaagccgaggacgacgccacctactattgccagcagtggtctaagcaccctctgacctttggctccggcaccaaggtggaaatcaagcgtacggtggctgcaccatctgtcttcatcttcccgccatctgatgagcagttgaaatctggtaccgctagcgttgtgtgcctgctgaataacttttatccacgggaggctaaggtgcagtggaaagtggacaatgccctccagagcggaaatagccaagagtccgttaccgaacaggactctaaagactctacatactccctgtcctccacactgaccctctccaaggccgactatgagaaacacaaggtttacgcatgcgaggtcacacaccagggactctcctctcccgtgaccaagagcttcaaccggggagaatgc

SEQ ID NO: 75 - protein, 449 aa, Artificial Sequence
  A-mab-Fc9
QVQLQQSGPELEKPGASVKISCKASGYSFTGYTMNWVKQSHGKSLEWIGLITPYNGASSYNQKFRGKATLTVDKSSSTAYMDLLSLTSEDSAVYFCARGGYDGRGFDYWGSGTPVTVSSASTKGPSVFPLAPSSKSTSGGTAALGCLVKDYFPEPVTVSWNSGALTSGVHTFPAVLQSSGLYSLSSVVTVPSSSLGTQTYICNVNHKPSNTKVDKRVEPKSCDKTHTCPPCPAPELLGGPSVFLFPPKPKDTLMISRTPEVTCVVVDVSHEDPEVKFNWYVDGVEVHNAKTKPREEQYNSTYRVVSVLTVLHQDWLNGKEYKCKVSNKALPAPIEKTISKAKGQPREPQVYTLPPSRDELTKNQVSLWCLVKGFYPSDIAVEWESNGQPENNYKTTPPVLDSDGSFFLYSALTVDKSRWQQGNVFSCSVMHEALHNHYTQKSLSLSPGK

SEQ ID NO: 76 - DNA, 1347 bp, Artificial Sequence
  nucleic acid molecules encoding A-mab-Fc9
caggttcagctgcagcagtctggacccgagctggaaaaacctggcgcctccgtgaagatcagctgcaaggccagcggctacagcttcaccggctacaccatgaactgggtcaagcagagccacggcaagagcctggaatggatcggcctgatcaccccttacaatggcgccagcagctacaaccagaagttcagaggcaaggccacactgaccgtggacaagagcagcagcaccgcctacatggatctgctgagcctgaccagcgaggacagcgccgtgtacttttgtgccagaggcggctatgacggcagaggctttgattactggggcagcggaacccctgtgaccgtttcttctgccagcactaaggggccctctgtgtttccactcgccccttctagcaaaagcacttccggaggaactgccgctctgggctgtctggtgaaagattacttccccgaaccagtcactgtgtcatggaactctggagcactgacatctggagttcacacctttcctgctgtgctgcagagttctggactgtactccctgtcatctgtggtcaccgtgccatcttcatctctggggacccagacctacatctgtaacgtgaaccacaaaccctccaacacaaaagtggacaaacgagtcgaaccaaaatcttgtgacaaaacccacacatgcccaccgtgcccagctccggaactcctgggcggaccgtcagtcttcctcttccccccaaaacccaaggacaccctcatgatctcccggacccctgaggtcacatgcgtggtggtggacgtgagccacgaagaccctgaggtcaagttcaactggtacgtggacggcgtggaggtgcataatgccaagacaaagccgcgggaggagcagtacaacagcacgtaccgtgtggtcagcgtcctcaccgtcctgcaccaggactggctgaatggcaaggagtacaagtgcaaggtctccaacaaagccctcccagcccccatcgagaaaaccatctccaaagccaaagggcagccccgagaaccacaggtgtacaccctgcccccaagtcgggatgagctgaccaagaaccaggtcagcctgtggtgcctggtcaaaggcttctatcccagcgacatcgccgtggagtgggagagcaatgggcagccggagaacaactacaagaccacgcctcccgtgttggactccgacggctccttcttcctctacagcgcgctcaccgtggacaagagcaggtggcagcaggggaacgtcttctcatgctccgtgatgcatgaggctctgcacaaccactacacgcagaagagcctctccctgtctccgggtaaa

SEQ ID NO: 77 - protein, 423 aa, Artificial Sequence
  muIFNa4-Fc6
MARLCAFLMILVMMSYYWSACSLGCDLPHTYNLGNKRALTVLEEMRRLPPLSCLKDRKDFGFPLEKVDNQQIQKAQAILVLRDLTQQILNLFTSKDLSATWNATLLDSFCNDLHQQLNDLKACVMQEPPLTQEDSLLAVRTYFHRITVYLRKKKHSLCAWEVIRAEVWRALSSSTNLLARLSEEKEGGGGSEPKSSDKTHTCPPCPAPELLGGPSVFLFPPKPKDTLMISRTPEVTCVVVDVSHEDPEVKFNWYVDGVEVHNAKTKPREEQYNSTYRVVSVLTVLHQDWLNGKEYKCKVSNKALPAPIEKTISKAKGQPREPQVYTLPPSRDELTKNQVSLSCGVKGFYPSDIAVEWESNGQPENNYKTTPPVLDSDGSFKLASKLTVDKSRWQQGNVFSCSVMHEALHNHYTQKSLSLSPGK

SEQ ID NO: 78 - DNA, 1269 bp, Artificial Sequence
  nucleic acid molecules encoding muIFNa4-Fc6
atggctaggctctgtgctttcctcatgatcctggtaatgatgagctactactggtcagcctgttctctaggatgtgacctgcctcacacttataacctcgggaacaagagggccttgacagtcctggaagaaatgagaagactcccccctctttcctgcctgaaggacaggaaggattttggattccccttggagaaggtggataaccaacagatccagaaggctcaagccatccttgtgctaagagatcttacccagcagattttgaacctcttcacatcaaaagacttgtctgctacttggaatgcaactctactagactcattctgcaatgacctccatcagcagctcaatgacctcaaagcctgtgtgatgcaggaacctcctctgacccaggaagactccctgctggctgtgaggacatacttccacaggatcactgtgtacctgagaaagaagaaacacagcctctgtgcctgggaggtgatcagagcagaagtctggagagccctctcttcctcaaccaacttgctggcaagactgagtgaggagaaggagggaggaggaggaagcgaacctaagagcagcgacaagacccacacttgccccccttgtcccgctccggaactcctgggcggaccgtcagtcttcctcttccccccaaaacccaaggacaccctcatgatctcccggacccctgaggtcacatgcgtggtggtggacgtgagccacgaagaccctgaggtcaagttcaactggtacgtggacggcgtggaggtgcataatgccaagacaaagccgcgggaggagcagtacaacagcacgtaccgtgtggtcagcgtcctcaccgtcctgcaccaggactggctgaatggcaaggagtacaagtgcaaggtctccaacaaagccctcccagcccccatcgagaaaaccatctccaaagccaaagggcagccccgagaaccacaggtgtataccctgcccccatcccgggatgagctgaccaagaaccaggtcagcctgagttgcggggtcaaaggcttctatcccagcgacatcgccgtggagtgggagagcaatgggcagccggagaacaactacaagaccacgcctcccgtgttggactccgacggctccttcaagctcgccagcaagctcaccgtggacaagagcaggtggcagcaggggaacgtcttctcatgctccgtgatgcatgaggctctgcacaaccactacacgcagaagagcctctccctgtctccgggtaaa

SEQ ID NO: 79 - protein, 5 aa, Artificial Sequence
  linker sequence
GSGGG

SEQ ID NO: 80 - protein, 425 aa, Artificial Sequence
  huIFNa2-Fc6
MALTFALLVALLVLSCKSSCSVGCDLPQTHSLGSRRTLMLLAQMRRISLFSCLKDRHDFGFPQEEFGNQFQKAETIPVLHEMIQQIFNLFSTKDSSAAWDETLLDKFYTELYQQLNDLEACVIQGVGVTETPLMKEDSILAVRKYFQRITLYLKEKKYSPCAWEVVRAEIMRSFSLSTNLQESLRSKEGGGGSEPKSSDKTHTCPPCPAPELLGGPSVFLFPPKPKDTLMISRTPEVTCVVVDVSHEDPEVKFNWYVDGVEVHNAKTKPREEQYNSTYRVVSVLTVLHQDWLNGKEYKCKVSNKALPAPIEKTISKAKGQPREPQVYTLPPSRDELTKNQVSLSCGVKGFYPSDIAVEWESNGQPENNYKTTPPVLDSDGSFKLASKLTVDKSRWQQGNVFSCSVMHEALHNHYTQKSLSLSPGK

SEQ ID NO: 81 - DNA, 1275 bp, Artificial Sequence
  nucleic acid molecules encoding huIFNa2-Fc6
atggccttgacctttgctttactggtggccctcctggtgctcagctgcaagtcaagctgctctgtgggctgtgatctgcctcaaacccacagcctgggtagcaggaggaccttgatgctcctggcacagatgaggagaatctctcttttctcctgcttgaaggacagacatgactttggatttccccaggaggagtttggcaaccagttccaaaaggctgaaaccatccctgtcctccatgagatgatccagcagatcttcaatctcttcagcacaaaggactcatctgctgcttgggatgagaccctcctagacaaattctacactgaactctaccagcagctgaatgacctggaagcctgtgtgatacagggggtgggggtgacagagactcccctgatgaaggaggactccattctggctgtgaggaaatacttccaaagaatcactctctatctgaaagagaagaaatacagcccttgtgcctgggaggttgtcagagcagaaatcatgagatctttttctttgtcaacaaacttgcaagaaagtttaagaagtaaggaaggaggaggaggaagcgaacctaagagcagcgacaagacccacacttgccccccttgtcccgctccggaactcctgggcggaccgtcagtcttcctcttccccccaaaacccaaggacaccctcatgatctcccggacccctgaggtcacatgcgtggtggtggacgtgagccacgaagaccctgaggtcaagttcaactggtacgtggacggcgtggaggtgcataatgccaagacaaagccgcgggaggagcagtacaacagcacgtaccgtgtggtcagcgtcctcaccgtcctgcaccaggactggctgaatggcaaggagtacaagtgcaaggtctccaacaaagccctcccagcccccatcgagaaaaccatctccaaagccaaagggcagccccgagaaccacaggtgtataccctgcccccatcccgggatgagctgaccaagaaccaggtcagcctgagttgcggggtcaaaggcttctatcccagcgacatcgccgtggagtgggagagcaatgggcagccggagaacaactacaagaccacgcctcccgtgttggactccgacggctccttcaagctcgccagcaagctcaccgtggacaagagcaggtggcagcaggggaacgtcttctcatgctccgtgatgcatgaggctctgcacaaccactacacgcagaagagcctctccctgtctccgggtaaa

SEQ ID NO: 82 - protein, 419 aa, Artificial Sequence
  muIFNb-Fc6
MNNRWILHAAFLLCFSTTALSINYKQLQLQERTNIRKCQELLEQLNGKINLTYRADFKIPMEMTEKMQKSYTAFAIQEMLQNVFLVFRNNFSSTGWNETIVVRLLDELHQQTVFLKTVLEEKQEERLTWEMSSTALHLKSYYWRVQRYLKLMKYNSYAWMVVRAEIFRNFLIIRRLTRNFQNGGGGSEPKSSDKTHTCPPCPAPELLGGPSVFLFPPKPKDTLMISRTPEVTCVVVDVSHEDPEVKFNWYVDGVEVHNAKTKPREEQYNSTYRVVSVLTVLHQDWLNGKEYKCKVSNKALPAPIEKTISKAKGQPREPQVYTLPPSRDELTKNQVSLSCGVKGFYPSDIAVEWESNGQPENNYKTTPPVLDSDGSFKLASKLTVDKSRWQQGNVFSCSVMHEALHNHYTQKSLSLSPGK

SEQ ID NO: 83 - DNA, 1257 bp, Artificial Sequence
  nucleic acid molecules encoding muIFNb-Fc6
atgaacaacaggtggattctccacgctgcgttcctgctgtgcttctccaccacagccctctccatcaactataagcagctccagctccaagaaaggacgaacattcggaaatgtcaggagctcctggagcagctgaatggaaagatcaacctcacctacagggcggacttcaagatccctatggagatgacggagaagatgcagaagagttacactgcctttgccatccaagagatgctccagaatgtctttcttgtcttcagaaacaatttctccagcactgggtggaatgagactattgttgtacgtctcctggatgaactccaccagcagacagtgtttctgaagacagtactagaggaaaagcaagaggaaagattgacgtgggagatgtcctcaactgctctccacttgaagagctattactggagggtgcaaaggtatcttaaactcatgaagtacaacagctacgcctggatggtggtccgagcagagatcttcaggaactttctcatcattcgaagacttaccagaaacttccaaaacggaggaggaggaagcgaacctaagagcagcgacaagacccacacttgccccccttgtcccgctccggaactcctgggcggaccgtcagtcttcctcttccccccaaaacccaaggacaccctcatgatctcccggacccctgaggtcacatgcgtggtggtggacgtgagccacgaagaccctgaggtcaagttcaactggtacgtggacggcgtggaggtgcataatgccaagacaaagccgcgggaggagcagtacaacagcacgtaccgtgtggtcagcgtcctcaccgtcctgcaccaggactggctgaatggcaaggagtacaagtgcaaggtctccaacaaagccctcccagcccccatcgagaaaaccatctccaaagccaaagggcagccccgagaaccacaggtgtataccctgcccccatcccgggatgagctgaccaagaaccaggtcagcctgagttgcggggtcaaaggcttctatcccagcgacatcgccgtggagtgggagagcaatgggcagccggagaacaactacaagaccacgcctcccgtgttggactccgacggctccttcaagctcgccagcaagctcaccgtggacaagagcaggtggcagcaggggaacgtcttctcatgctccgtgatgcatgaggctctgcacaaccactacacgcagaagagcctctccctgtctccgggtaaa

SEQ ID NO: 84 - protein, 424 aa, Artificial Sequence
  huIFNb-Fc6
MTNKCLLQIALLLCFSTTALSMSYNLLGFLQRSSNFQCQKLLWQLNGRLEYCLKDRMNFDIPEEIKQLQQFQKEDAALTIYEMLQNIFAIFRQDSSSTGWNETIVENLLANVYHQINHLKTVLEEKLEKEDFTRGKLMSSLHLKRYYGRILHYLKAKEYSHCAWTIVRVEILRNFYFINRLTGYLRNGGGGSEPKSSDKTHTCPPCPAPELLGGPSVFLFPPKPKDTLMISRTPEVTCVVVDVSHEDPEVKFNWYVDGVEVHNAKTKPREEQYNSTYRVVSVLTVLHQDWLNGKEYKCKVSNKALPAPIEKTISKAKGQPREPQVYTLPPSRDELTKNQVSLSCGVKGFYPSDIAVEWESNGQPENNYKTTPPVLDSDGSFKLASKLTVDKSRWQQGNVFSCSVMHEALHNHYTQKSLSLSPGK

SEQ ID NO: 85 - DNA, 1272 bp, Artificial Sequence
  nucleic acid molecules encoding huIFNb-Fc6
ttggattcctacaaagaagcagcaattttcagtgtcagaagctcctgtggcaattgaatgggaggcttgaatactgcctcaaggacaggatgaactttgacatccctgaggagattaagcagctgcagcagttccagaaggaggacgccgcattgaccatctatgagatgctccagaacatctttgctattttcagacaagattcatctagcactggctggaatgagactattgttgagaacctcctggctaatgtctatcatcagataaaccatctgaagacagtcctggaagaaaaactggagaaagaagatttcaccaggggaaaactcatgagcagtctgcacctgaaaagatattatgggaggattctgcattacctgaaggccaaggagtacagtcactgtgcctggaccatagtcagagtggaaatcctaaggaacttttacttcattaacagacttacaggttacctccgaaacggatccggtggaggtgacaagacccacacctgccccccctgccccgcccccgagctgctgggcggccccagcgtgttccggaggaggaggaagcgaacctaagagcagcgacaagacccacacttgccccccttgtcccgctccggaactcctgggcggaccgtcagtcttcctcttccccccaaaacccaaggacaccctcatgatctcccggacccctgaggtcacatgcgtggtggtggacgtgagccacgaagaccctgaggtcaagttcaactggtacgtggacggcgtggaggtgcataatgccaagacaaagccgcgggaggagcagtacaacagcacgtaccgtgtggtcagcgtcctcaccgtcctgcaccaggactggctgaatggcaaggagtacaagtgcaaggtctccaacaaagccctcccagcccccatcgagaaaaccatctccaaagccaaagggcagccccgagaaccacaggtgtataccctgcccccatcccgggatgagctgaccaagaaccaggtcagcctgagttgcggggtcaaaggcttctatcccagcgacatcgccgtggagtgggagagcaatgggcagccggagaacaactacaagaccacgcctcccgtgttggactccgacggctccttcaagctcgccagcaagctcaccgtggacaagagcaggtggcagcaggggaacgtcttctcatgctccgtgatgcatgaggctctgcacaaccactacacgcagaagagcctctccctgtctccgggtaaa

SEQ ID NO: 86 - protein, 437 aa, Artificial Sequence
  huIFNL-Fc6
MAAAWTVVLVTLVLGLAVAGPVPTSKPTTTGKGCHIGRFKSLSPQELASFKKARDALEESLKLKNWSCSSPVFPGNWDLRLLQVRERPVALEAELALTLKVLEAAAGPALEDVLDQPLHTLHHILSQLQACIQPQPTAGPRPRGRLHHWLHRLQEAPKKESAGCLEASVTFNLFRLLTRDLKYVADGNLCLRTSTHPESTGGGGSEPKSSDKTHTCPPCPAPELLGGPSVFLFPPKPKDTLMISRTPEVTCVVVDVSHEDPEVKFNWYVDGVEVHNAKTKPREEQYNSTYRVVSVLTVLHQDWLNGKEYKCKVSNKALPAPIEKTISKAKGQPREPQVYTLPPSRDELTKNQVSLSCGVKGFYPSDIAVEWESNGQPENNYKTTPPVLDSDGSFKLASKLTVDKSRWQQGNVFSCSVMHEALHNHYTQKSLSLSPGK

SEQ ID NO: 87 - DNA, 1311 bp, Artificial Sequence
  nucleic acid molecules encoding huIFNL-Fc6
atggctgcagcttggaccgtggtgctggtgactttggtgctaggcttggccgtggcaggccctgtccccacttccaagcccaccacaactgggaagggctgccacattggcaggttcaaatctctgtcaccacaggagctagcgagcttcaagaaggccagggacgccttggaagagtcactcaagctgaaaaactggagttgcagctctcctgtcttccccgggaattgggacctgaggcttctccaggtgagggagcgccctgtggccttggaggctgagctggccctgacgctgaaggtcctggaggccgctgctggcccagccctggaggacgtcctagaccagccccttcacaccctgcaccacatcctctcccagctccaggcctgtatccagcctcagcccacagcagggcccaggccccggggccgcctccaccactggctgcaccggctccaggaggcccccaaaaaggagtccgctggctgcctggaggcatctgtcaccttcaacctcttccgcctcctcacgcgagacctcaaatatgtggccgatgggaacctgtgtctgagaacgtcaacccaccctgagtccaccggaggaggaggaagcgaacctaagagcagcgacaagacccacacttgccccccttgtcccgctccggaactcctgggcggaccgtcagtcttcctcttccccccaaaacccaaggacaccctcatgatctcccggacccctgaggtcacatgcgtggtggtggacgtgagccacgaagaccctgaggtcaagttcaactggtacgtggacggcgtggaggtgcataatgccaagacaaagccgcgggaggagcagtacaacagcacgtaccgtgtggtcagcgtcctcaccgtcctgcaccaggactggctgaatggcaaggagtacaagtgcaaggtctccaacaaagccctcccagcccccatcgagaaaaccatctccaaagccaaagggcagccccgagaaccacaggtgtataccctgcccccatcccgggatgagctgaccaagaaccaggtcagcctgagttgcggggtcaaaggcttctatcccagcgacatcgccgtggagtgggagagcaatgggcagccggagaacaactacaagaccacgcctcccgtgttggactccgacggctccttcaagctcgccagcaagctcaccgtggacaagagcaggtggcagcaggggaacgtcttctcatgctccgtgatgcatgaggctctgcacaaccactacacgcagaagagcctctccctgtctccgggtaaa

SEQ ID NO: 88 - protein, 15 aa, Artificial Sequence
  linker sequence
GGGGSGGGGSGGGGS

SEQ ID NO: 89 - protein, 407 aa, Artificial Sequence
  huIL10-Fc6
SPGQGTQSENSCTHFPGNLPNMLRDLRDAFSRVKTFFQMKDQLDNLLLKESLLEDFKGYLGCQALSEMIQFYLEEVMPQAENQDPDIKAHVNSLGENLKTLRLRLRRCHRFLPCENKSKAVEQVKNAFNKLQEKGIYKAMSEFDIFINYIEAYMTMKIRNGGGGSGGGGSGGGGSEPKSSDKTHTCPPCPAPELLGGPSVFLFPPKPKDTLMISRTPEVTCVVVDVSHEDPEVKFNWYVDGVEVHNAKTKPREEQYNSTYRVVSVLTVLHQDWLNGKEYKCKVSNKALPAPIEKTISKAKGQPREPQVYTLPPSRDELTKNQVSLSCGVKGFYPSDIAVEWESNGQPENNYKTTPPVLDSDGSFKLASKLTVDKSRWQQGNVFSCSVMHEALHNHYTQKSLSLSPGK

SEQ ID NO: 90 - DNA, 1221 bp, Artificial Sequence
  nucleic acid molecules encoding huIL10-Fc6
agccccggccagggcacacagtccgagaacagctgcacccactttcccggcaacctgcctaacatgctgagggacctgagggacgccttcagcagggtgaagaccttcttccagatgaaggaccagctggataacctgctgctgaaggagagcctgctggaggacttcaagggctacctgggctgccaggccctgagcgagatgatccagttctacctggaggaggtgatgccccaggccgagaaccaggaccccgacatcaaggcccacgtgaacagcctgggcgagaacctgaagaccctgaggctgaggctgaggaggtgccacaggttcctgccctgtgagaacaaatccaaggccgtggagcaggtgaagaacgccttcaacaagctgcaggaaaagggcatctacaaggccatgagcgagttcgacatctttatcaactatatcgaggcctacatgacaatgaagatcaggaacggcggcggcggcagcgggggcggcggcagcggaggaggcggcagcgaacctaagagcagcgacaagacccacacttgccccccttgtcccgctccggaactcctgggcggaccgtcagtcttcctcttccccccaaaacccaaggacaccctcatgatctcccggacccctgaggtcacatgcgtggtggtggacgtgagccacgaagaccctgaggtcaagttcaactggtacgtggacggcgtggaggtgcataatgccaagacaaagccgcgggaggagcagtacaacagcacgtaccgtgtggtcagcgtcctcaccgtcctgcaccaggactggctgaatggcaaggagtacaagtgcaaggtctccaacaaagccctcccagcccccatcgagaaaaccatctccaaagccaaagggcagccccgagaaccacaggtgtataccctgcccccatcccgggatgagctgaccaagaaccaggtcagcctgagttgcggggtcaaaggcttctatcccagcgacatcgccgtggagtgggagagcaatgggcagccggagaacaactacaagaccacgcctcccgtgttggactccgacggctccttcaagctcgccagcaagctcaccgtggacaagagcaggtggcagcaggggaacgtcttctcatgctccgtgatgcatgaggctctgcacaaccactacacgcagaagagcctctccctgtctccgggtaaa

SEQ ID NO: 91 - protein, 582 aa, Artificial Sequence
  (huIL10)2-Fc6
SPGQGTQSENSCTHFPGNLPNMLRDLRDAFSRVKTFFQMKDQLDNLLLKESLLEDFKGYLGCQALSEMIQFYLEEVMPQAENQDPDIKAHVNSLGENLKTLRLRLRRCHRFLPCENKSKAVEQVKNAFNKLQEKGIYKAMSEFDIFINYIEAYMTMKIRNGGGGSGGGGSGGGGSSPGQGTQSENSCTHFPGNLPNMLRDLRDAFSRVKTFFQMKDQLDNLLLKESLLEDFKGYLGCQALSEMIQFYLEEVMPQAENQDPDIKAHVNSLGENLKTLRLRLRRCHRFLPCENKSKAVEQVKNAFNKLQEKGIYKAMSEFDIFINYIEAYMTMKIRNGGGGSGGGGSGGGGSEPKSSDKTHTCPPCPAPELLGGPSVFLFPPKPKDTLMISRTPEVTCVVVDVSHEDPEVKFNWYVDGVEVHNAKTKPREEQYNSTYRVVSVLTVLHQDWLNGKEYKCKVSNKALPAPIEKTISKAKGQPREPQVYTLPPSRDELTKNQVSLSCGVKGFYPSDIAVEWESNGQPENNYKTTPPVLDSDGSFKLASKLTVDKSRWQQGNVFSCSVMHEALHNHYTQKSLSLSPGK

SEQ ID NO: 92 - DNA, 1746 bp, Artificial Sequence
  nucleic acid molecules encoding (huIL10)2-Fc6
agccccggccagggcacacagtccgagaacagctgcacccactttcccggcaacctgcctaacatgctgagggacctgagggacgccttcagcagggtgaagaccttcttccagatgaaggaccagctggataacctgctgctgaaggagagcctgctggaggacttcaagggctacctgggctgccaggccctgagcgagatgatccagttctacctggaggaggtgatgccccaggccgagaaccaggaccccgacatcaaggcccacgtgaacagcctgggcgagaacctgaagaccctgaggctgaggctgaggaggtgccacaggttcctgccctgtgagaacaaatccaaggccgtggagcaggtgaagaacgccttcaacaagctgcaggaaaagggcatctacaaggccatgagcgagttcgacatctttatcaactatatcgaggcctacatgacaatgaagatcaggaacggcggcggcggcagcgggggcggcggcagcggaggaggcggcagcagccccggccagggcacacagtccgagaacagctgcacccactttcccggcaacctgcctaacatgctgagggacctgagggacgccttcagcagggtgaagaccttcttccagatgaaggaccagctggataacctgctgctgaaggagagcctgctggaggacttcaagggctacctgggctgccaggccctgagcgagatgatccagttctacctggaggaggtgatgccccaggccgagaaccaggaccccgacatcaaggcccacgtgaacagcctgggcgagaacctgaagaccctgaggctgaggctgaggaggtgccacaggttcctgccctgtgagaacaaatccaaggccgtggagcaggtgaagaacgccttcaacaagctgcaggaaaagggcatctacaaggccatgagcgagttcgacatctttatcaactatatcgaggcctacatgacaatgaagatcaggaacggcggcggcggcagcgggggcggcggcagcggaggaggcggcagcgaacctaagagcagcgacaagacccacacttgccccccttgtcccgctccggaactcctgggcggaccgtcagtcttcctcttccccccaaaacccaaggacaccctcatgatctcccggacccctgaggtcacatgcgtggtggtggacgtgagccacgaagaccctgaggtcaagttcaactggtacgtggacggcgtggaggtgcataatgccaagacaaagccgcgggaggagcagtacaacagcacgtaccgtgtggtcagcgtcctcaccgtcctgcaccaggactggctgaatggcaaggagtacaagtgcaaggtctccaacaaagccctcccagcccccatcgagaaaaccatctccaaagccaaagggcagccccgagaaccacaggtgtataccctgcccccatcccgggatgagctgaccaagaaccaggtcagcctgagttgcggggtcaaaggcttctatcccagcgacatcgccgtggagtgggagagcaatgggcagccggagaacaactacaagaccacgcctcccgtgttggactccgacggctccttcaagctcgccagcaagctcaccgtggacaagagcaggtggcagcaggggaacgtcttctcatgctccgtgatgcatgaggctctgcacaaccactacacgcagaagagcctctccctgtctccgggtaaa

SEQ ID NO: 93 - protein, 577 aa, Artificial Sequence
  (huIL10)2-Fc9
SPGQGTQSENSCTHFPGNLPNMLRDLRDAFSRVKTFFQMKDQLDNLLLKESLLEDFKGYLGCQALSEMIQFYLEEVMPQAENQDPDIKAHVNSLGENLKTLRLRLRRCHRFLPCENKSKAVEQVKNAFNKLQEKGIYKAMSEFDIFINYIEAYMTMKIRNGGGGSGGGGSGGGGSSPGQGTQSENSCTHFPGNLPNMLRDLRDAFSRVKTFFQMKDQLDNLLLKESLLEDFKGYLGCQALSEMIQFYLEEVMPQAENQDPDIKAHVNSLGENLKTLRLRLRRCHRFLPCENKSKAVEQVKNAFNKLQEKGIYKAMSEFDIFINYIEAYMTMKIRNGGGGSGGGGSGGGGSDKTHTCPPCPAPELLGGPSVFLFPPKPKDTLMISRTPEVTCVVVDVSHENPEVKFNWYVDGVEVHNAKTKPREEQYNSTYRVVSVLTVLHQDWLNGKEYKCKVSNKALPAPIEKTISKAKGQPREPQVYTLPPSRDELTKNQVSLWCLVKGFYPSDIAVEWESNGQPENNYKTTPPVLDSDGSFFLYSALTVDKSRWQQGNVFSCSVMHEALHNHYTQKSLSLSPGK

SEQ ID NO: 94 - DNA, 1731 bp, Artificial Sequence
  nucleic acid molecules encoding (huIL10)2-Fc9
agccccggccagggcacacagtccgagaacagctgcacccactttcccggcaacctgcctaacatgctgagggacctgagggacgccttcagcagggtgaagaccttcttccagatgaaggaccagctggataacctgctgctgaaggagagcctgctggaggacttcaagggctacctgggctgccaggccctgagcgagatgatccagttctacctggaggaggtgatgccccaggccgagaaccaggaccccgacatcaaggcccacgtgaacagcctgggcgagaacctgaagaccctgaggctgaggctgaggaggtgccacaggttcctgccctgtgagaacaaatccaaggccgtggagcaggtgaagaacgccttcaacaagctgcaggaaaagggcatctacaaggccatgagcgagttcgacatctttatcaactatatcgaggcctacatgacaatgaagatcaggaacggcggcggcggcagcgggggcggcggcagcggaggaggcggcagcagccccggccagggcacacagtccgagaacagctgcacccactttcccggcaacctgcctaacatgctgagggacctgagggacgccttcagcagggtgaagaccttcttccagatgaaggaccagctggataacctgctgctgaaggagagcctgctggaggacttcaagggctacctgggctgccaggccctgagcgagatgatccagttctacctggaggaggtgatgccccaggccgagaaccaggaccccgacatcaaggcccacgtgaacagcctgggcgagaacctgaagaccctgaggctgaggctgaggaggtgccacaggttcctgccctgtgagaacaaatccaaggccgtggagcaggtgaagaacgccttcaacaagctgcaggaaaagggcatctacaaggccatgagcgagttcgacatctttatcaactatatcgaggcctacatgacaatgaagatcaggaacggcggcggcggcagcgggggcggcggcagcggaggaggcggcagcgacaaaacccacacatgcccaccgtgcccagctccggaactcctgggcggaccgtcagtcttcctcttccccccaaaacccaaggacaccctcatgatctcccggacccctgaggtcacatgcgtggtggtggacgtgagccacgaagaccctgaggtcaagttcaactggtacgtggacggcgtggaggtgcataatgccaagacaaagccgcgggaggagcagtacaacagcacgtaccgtgtggtcagcgtcctcaccgtcctgcaccaggactggctgaatggcaaggagtacaagtgcaaggtctccaacaaagccctcccagcccccatcgagaaaaccatctccaaagccaaagggcagccccgagaaccacaggtgtacaccctgcccccaagtcgggatgagctgaccaagaaccaggtcagcctgtggtgcctggtcaaaggcttctatcccagcgacatcgccgtggagtgggagagcaatgggcagccggagaacaactacaagaccacgcctcccgtgttggactccgacggctccttcttcctctacagcgcgctcaccgtggacaagagcaggtggcagcaggggaacgtcttctcatgctccgtgatgcatgaggctctgcacaaccactacacgcagaagagcctctccctgtctccgggtaaa

SEQ ID NO: 95 - protein, 577 aa, Artificial Sequence
  (huIL10)2-Fc-hole
SPGQGTQSENSCTHFPGNLPNMLRDLRDAFSRVKTFFQMKDQLDNLLLKESLLEDFKGYLGCQALSEMIQFYLEEVMPQAENQDPDIKAHVNSLGENLKTLRLRLRRCHRFLPCENKSKAVEQVKNAFNKLQEKGIYKAMSEFDIFINYIEAYMTMKIRNGGGGSGGGGSGGGGSSPGQGTQSENSCTHFPGNLPNMLRDLRDAFSRVKTFFQMKDQLDNLLLKESLLEDFKGYLGCQALSEMIQFYLEEVMPQAENQDPDIKAHVNSLGENLKTLRLRLRRCHRFLPCENKSKAVEQVKNAFNKLQEKGIYKAMSEFDIFINYIEAYMTMKIRNGGGGSGGGGSGGGGSDKTHTCPPCPAPELLGGPSVFLFPPKPKDTLMISRTPEVTCVVVDVSHEDPEVKFNWYVDGVEVHNAKTKPREEQYNSTYRVVSVLTVLHQDWLNGKEYKCKVSNKALPAPIEKTISKAKGQPREPQVCTLPPSRDELTKNQVSLSCAVKGFYPSDIAVEWESNGQPENNYKTTPPVLDSDGSFFLVSKLTVDKSRWQQGNVFSCSVMHEALHNHYTQKSLSLSPGK

SEQ ID NO: 96 - DNA, 1731 bp, Artificial Sequence
  nucleic acid molecules encoding (huIL10)2-Fc-hole
agccccggccagggcacacagtccgagaacagctgcacccactttcccggcaacctgcctaacatgctgagggacctgagggacgccttcagcagggtgaagaccttcttccagatgaaggaccagctggataacctgctgctgaaggagagcctgctggaggacttcaagggctacctgggctgccaggccctgagcgagatgatccagttctacctggaggaggtgatgccccaggccgagaaccaggaccccgacatcaaggcccacgtgaacagcctgggcgagaacctgaagaccctgaggctgaggctgaggaggtgccacaggttcctgccctgtgagaacaaatccaaggccgtggagcaggtgaagaacgccttcaacaagctgcaggaaaagggcatctacaaggccatgagcgagttcgacatctttatcaactatatcgaggcctacatgacaatgaagatcaggaacggcggcggcggcagcgggggcggcggcagcggaggaggcggcagcagccccggccagggcacacagtccgagaacagctgcacccactttcccggcaacctgcctaacatgctgagggacctgagggacgccttcagcagggtgaagaccttcttccagatgaaggaccagctggataacctgctgctgaaggagagcctgctggaggacttcaagggctacctgggctgccaggccctgagcgagatgatccagttctacctggaggaggtgatgccccaggccgagaaccaggaccccgacatcaaggcccacgtgaacagcctgggcgagaacctgaagaccctgaggctgaggctgaggaggtgccacaggttcctgccctgtgagaacaaatccaaggccgtggagcaggtgaagaacgccttcaacaagctgcaggaaaagggcatctacaaggccatgagcgagttcgacatctttatcaactatatcgaggcctacatgacaatgaagatcaggaacggcggcggcggcagcgggggcggcggcagcggaggaggcggcagcgacaagacccacacctgccccccttgccccgctccggagctgctgggcggccccagcgtgttcctgttcccccccaagcccaaggacaccctgatgatcagccgcacccccgaggtgacctgcgtggtggtggacgtgagccacgaggaccccgaggtgaagttcaactggtacgtggacggcgtggaggtgcacaacgccaagaccaagccccgcgaggagcagtacaacagcacctaccgcgtggtgagcgtgctgaccgtgctgcaccaggactggctgaacggcaaggagtacaagtgcaaggtgagcaacaaggccctgcccgcccccatcgagaagaccatcagcaaggccaagggccagccccgcgagccccaggtgtgcaccctgccccccagccgcgacgagctgaccaagaaccaggtgagcctgagctgcgccgtgaagggcttctaccccagcgacatcgccgtggagtgggagagcaacggccagcccgagaacaactacaagaccaccccccccgtgctggacagcgacggcagcttcttcctggtgagcaagctgaccgtggacaagagccgctggcagcagggcaacgtgttcagctgcagcgtgatgcacgaggccctgcacaaccactacacccagaagagcctgagcctgagccccggcaag

SEQ ID NO: 97 - protein, 370 aa, Artificial Sequence
  husIL2-Fc6
APTSSSTKKTQLQLEHLLLDLQMILNGINNYKNPKLTRMLTFKFYMPKKATELKHLQCLEEELKPLEEVLNLAQSKNFHFDPRDVVSNINVFVLELKGSETTFMCEYADETATIVEFLNRWITFCQSIISTLTGGGGSEPKSSDKTHTCPPCPAPELLGGPSVFLFPPKPKDTLMISRTPEVTCVVVDVSHEDPEVKFNWYVDGVEVHNAKTKPREEQYNSTYRVVSVLTVLHQDWLNGKEYKCKVSNKALPAPIEKTISKAKGQPREPQVYTLPPSRDELTKNQVSLSCGVKGFYPSDIAVEWESNGQPENNYKTTPPVLDSDGSFKLASKLTVDKSRWQQGNVFSCSVMHEALHNHYTQKSLSLSPGK

SEQ ID NO: 98 - DNA, 1110 bp, Artificial Sequence
  nucleic acid molecules encoding husIL2-Fc6
gcccctacaagcagcagcaccaagaagacccagctgcagctggaacacctgctgctggatctgcagatgatcctgaacggcatcaacaactacaagaaccccaagctgacccggatgctgaccttcaagttctacatgcccaagaaggccaccgagctgaagcacctccagtgtctggaggaggagctgaagcctctggaggaagtgctgaacctggcccagagcaagaacttccacttcgaccccagggacgtggtgtccaacatcaacgtgttcgtgctggaactgaagggcagcgagaccaccttcatgtgcgagtacgccgacgagaccgctaccatcgtggagttcctgaaccgctggatcaccttttgccagagcatcatcagcacactgaccggaggaggaggaagcgaacctaagagcagcgacaagacccacacttgccccccttgtcccgctccggaactcctgggcggaccgtcagtcttcctcttccccccaaaacccaaggacaccctcatgatctcccggacccctgaggtcacatgcgtggtggtggacgtgagccacgaagaccctgaggtcaagttcaactggtacgtggacggcgtggaggtgcataatgccaagacaaagccgcgggaggagcagtacaacagcacgtaccgtgtggtcagcgtcctcaccgtcctgcaccaggactggctgaatggcaaggagtacaagtgcaaggtctccaacaaagccctcccagcccccatcgagaaaaccatctccaaagccaaagggcagccccgagaaccacaggtgtataccctgcccccatcccgggatgagctgaccaagaaccaggtcagcctgagttgcggggtcaaaggcttctatcccagcgacatcgccgtggagtgggagagcaatgggcagccggagaacaactacaagaccacgcctcccgtgttggactccgacggctccttcaagctcgccagcaagctcaccgtggacaagagcaggtggcagcaggggaacgtcttctcatgctccgtgatgcatgaggctctgcacaaccactacacgcagaagagcctctccctgtctccgggtaaa

SEQ ID NO: 99 - protein, 370 aa, Artificial Sequence
  husIL2-Fc-hole
APTSSSTKKTQLQLEHLLLDLQMILNGINNYKNPKLTRMLTFKFYMPKKATELKHLQCLEEELKPLEEVLNLAQSKNFHFDPRDVVSNINVFVLELKGSETTFMCEYADETATIVEFLNRWITFCQSIISTLTGGGGSEPKSSDKTHTCPPCPAPELLGGPSVFLFPPKPKDTLMISRTPEVTCVVVDVSHEDPEVKFNWYVDGVEVHNAKTKPREEQYNSTYRVVSVLTVLHQDWLNGKEYKCKVSNKALPAPIEKTISKAKGQPREPQVYTLPPSRCELTKNQVSLSCAVKGFYPSDIAVEWESNGQPENNYKTTPPVLDSDGSFFLVSKLTVDKSRWQQGNVFSCSVMHEALHNHYTQKSLSLSPGK

SEQ ID NO: 100 - DNA, 1110 bp, Artificial Sequence
  nucleic acid molecules encoding husIL2-Fc-hole
gcccctacaagcagcagcaccaagaagacccagctgcagctggaacacctgctgctggatctgcagatgatcctgaacggcatcaacaactacaagaaccccaagctgacccggatgctgaccttcaagttctacatgcccaagaaggccaccgagctgaagcacctccagtgtctggaggaggagctgaagcctctggaggaagtgctgaacctggcccagagcaagaacttccacttcgaccccagggacgtggtgtccaacatcaacgtgttcgtgctggaactgaagggcagcgagaccaccttcatgtgcgagtacgccgacgagaccgctaccatcgtggagttcctgaaccgctggatcaccttttgccagagcatcatcagcacactgaccggaggaggaggaagcgagcctaagtccagcgacaagacccacacctgccccccttgccccgctccggaactcctgggcggaccgtcagtcttcctcttccccccaaaacccaaggacaccctcatgatctcccggacccctgaggtcacatgcgtggtggtggacgtgagccacgaagaccctgaggtcaagttcaactggtacgtggacggcgtggaggtgcataatgccaagacaaagccgcgggaggagcagtacaacagcacgtaccgtgtggtcagcgtcctcaccgtcctgcaccaggactggctgaatggcaaggagtacaagtgcaaggtctccaacaaagccctcccagcccccatcgagaaaaccatctccaaagccaaagggcagccccgagaaccacaggtgtataccctgcccccatcccggtgtgagctgaccaagaaccaggtcagcctgagttgcgcggtcaaaggcttctatcccagcgacatcgccgtggagtgggagagcaatgggcagccggagaacaactacaagaccacgcctcccgtgttggactccgacggctccttcttcctcgtcagcaagctcaccgtggacaagagcaggtggcagcaggggaacgtcttctcatgctccgtgatgcatgaggctctgcacaaccactacacgcagaagagcctctccctgtctccgggtaaa

SEQ ID NO: 101 - protein, 11 aa, Artificial Sequence
  Cetuximab light chain CDR1
RASQSIGTNIH

SEQ ID NO: 102 - protein, 7 aa, Artificial Sequence
  Cetuximab light chain CDR2
YASESIS

SEQ ID NO: 103 - protein, 9 aa, Artificial Sequence
  Cetuximab light chain CDR3
QQNNNWPTT

SEQ ID NO: 104 - protein, 107 aa, Artificial Sequence
  Cetuximab light chain variable region
DILLTQSPVILSVSPGERVSFSCRASQSIGTNIHWYQQRTNGSPRLLIKYASESISGIPSRFSGSGSGTDFTLSINSVESEDIADYYCQQNNNWPTTFGAGTKLELK

SEQ ID NO: 105 - protein, 5 aa, Artificial Sequence
  Cetuximab heavy chain CDR1
NYGVH

SEQ ID NO: 106 - protein, 16 aa, Artificial Sequence
  Cetuximab heavy chain CDR2
VIWSGGNTDYNTPFTS

SEQ ID NO: 107 - protein, 11 aa, Artificial Sequence
  Cetuximab heavy chain CDR3
ALTYYDYEFAY

SEQ ID NO: 108 - protein, 119 aa, Artificial Sequence
  Cetuximab heavy chain variable region
QVQLKQSGPGLVQPSQSLSITCTVSGFSLTNYGVHWVRQSPGKGLEWLGVIWSGGNTDYNTPFTSRLSINKDNSKSQVFFKMNSLQSNDTAIYYCARALTYYDYEFAYWGQGTLVTVSA

SEQ ID NO: 109 - protein, 11 aa, Artificial Sequence
  Mab806 light chain CDR1
HSSQDINSNIG

SEQ ID NO: 110 - protein, 7 aa, Artificial Sequence
  Mab806 light chain CDR2
HGTNLDD

SEQ ID NO: 111 - protein, 9 aa, Artificial Sequence
  Mab806 light chain CDR3
VQYAQFPWT

SEQ ID NO: 112 - protein, 107 aa, Artificial Sequence
  Mab806 light chain variable region
DILMTQSPSSMSVSLGDTVSITCHSSQDINSNIGWLQQRPGKSFKGLIYHGTNLDDEVPSRFSGSGSGADYSLTISSLESEDFADYYCVQYAQFPWTFGGGTKLEIK

SEQ ID NO: 113 - protein, 6 aa, Artificial Sequence
  Mab806 heavy chain CDR1
SDFAWN

SEQ ID NO: 114 - protein, 16 aa, Artificial Sequence
  Mab806 heavy chain CDR2
YISYSGNTRYNPSLKS

SEQ ID NO: 115 - protein, 7 aa, Artificial Sequence
  Mab806 heavy chain CDR3
AGRGFPY

SEQ ID NO: 116 - protein, 116 aa, Artificial Sequence
  Mab806 heavy chain variable region
DVQLQESGPSLVKPSQSLSLTCTVTGYSITSDFAWNWIRQFPGNKLEWMGYISYSGNTRYNPSLKSRISITRDTSKNQFFLQLNSVTIEDTATYYCVTAGRGFPYWGQGTLVTVSA

SEQ ID NO: 117 - protein, 11 aa, Artificial Sequence
  Trastuzumab light chain CDR1
RASQDVNTAVA

SEQ ID NO: 118 - protein, 7 aa, Artificial Sequence
  Trastuzumab light chain CDR2
SASFLYS

SEQ ID NO: 119 - protein, 9 aa, Artificial Sequence
  Trastuzumab light chain CDR3
QQHYTTPPT

SEQ ID NO: 120 - protein, 107 aa, Artificial Sequence [sequence omitted]

SEQ ID NO: 121 - protein, 5 aa, Artificial Sequence
  Trastuzumab heavy chain CDR1
DTYIH

SEQ ID NO: 122 - protein, 17 aa, Artificial Sequence
  Trastuzumab heavy chain CDR2
RIYPTNGYTRYADSVKG

SEQ ID NO: 123 - protein, 11 aa, Artificial Sequence
  Trastuzumab heavy chain CDR3
WGGDGFYAMDY

SEQ ID NO: 124 - protein, 120 aa, Artificial Sequence [sequence omitted]

SEQ ID NO: 125 - protein, 11 aa, Artificial Sequence
  Pertuzumab light chain CDR1
KASQDVSIGVA

SEQ ID NO: 126 - protein, 7 aa, Artificial Sequence
  Pertuzumab light chain CDR2
SASYRYT

SEQ ID NO: 127 - protein, 9 aa, Artificial Sequence
  Pertuzumab light chain CDR3
QQYYIYPYT

SEQ ID NO: 128 - protein, 107 aa, Artificial Sequence [sequence omitted]

SEQ ID NO: 129 - protein, 5 aa, Artificial Sequence
  Pertuzumab heavy chain CDR1
DYTMD

SEQ ID NO: 130 - protein, 17 aa, Artificial Sequence
  Pertuzumab heavy chain CDR2
DVNPNSGGSIYNQRFKG

SEQ ID NO: 131 - protein, 10 aa, Artificial Sequence
  Pertuzumab heavy chain CDR3
NLGPSFYFDY

SEQ ID NO: 132 - protein, 119 aa, Artificial Sequence [sequence omitted]

SEQ ID NO: 133 - protein, 16 aa, Artificial Sequence
  C-MAB light chain CDR1
RSSQSLVHSNRNTYLH

SEQ ID NO: 134 - protein, 7 aa, Artificial Sequence
  C-MAB light chain CDR2
KVSNRFS

SEQ ID NO: 135 - protein, 9 aa, Artificial Sequence
  C-MAB light chain CDR3
SQNTHVPPT

SEQ ID NO: 136 - protein, 112 aa, Artificial Sequence
  C-MAB light chain variable region
DVVMTQSPLSLPVTPGEPASISCRSSQSLVHSNRNTYLHWYLQKPGQSPQLLIYKVSNRFSGVPDRFSGSGSGTDFTLKISRVEAEDVGVYYCSQNTHVPPTFGQGTKLEIK

SEQ ID NO: 137 - protein, 5 aa, Artificial Sequence
  C-MAB heavy chain CDR1
DYEMH

SEQ ID NO: 138 - protein, 17 aa, Artificial Sequence
  C-MAB heavy chain CDR2
ALDPKTGDTAYSQKFKG

SEQ ID NO: 139 - protein, 6 aa, Artificial Sequence
  C-MAB heavy chain CDR3
FYSYTY

SEQ ID NO: 140 - protein, 115 aa, Artificial Sequence
  C-MAB heavy chain variable region
QVQLVQSGAEVKKPGASVKVSCKASGYTFTDYEMHWVRQAPGQGLEWMGALDPKTGDTAYSQKFKGRVTLTADKSTSTAYMELSSLTSEDTAVYYCTRFYSYTYWGQGTLVTVSS

SEQ ID NO: 141 - protein, 6 aa, Artificial Sequence
  28H1 light chain CDR1
SRSYLA

SEQ ID NO: 142 - protein, 7 aa, Artificial Sequence
  28H1 light chain CDR2
GASTRAT

SEQ ID NO: 143 - protein, 9 aa, Artificial Sequence
  28H1 light chain CDR3
QQGQVIPPT

SEQ ID NO: 144 - protein, 108 aa, Artificial Sequence
  28H1 light chain variable region
EIVLTQSPGTLSLSPGERATLSCRASQSVSRSYLAWYQQKPGQAPRLLIIGASTRATGIPDRFSGSGSGTDFTLTISRLEPEDFAVYYCQQGQVIPPTFGQGTKVEIK

SEQ ID NO: 145 - protein, 5 aa, Artificial Sequence
  28H1 heavy chain CDR1
SHAMS

SEQ ID NO: 146 - protein, 16 aa, Artificial Sequence
  28H1 heavy chain CDR2
AIWASGEQYYADSVKG

SEQ ID NO: 147 - protein, 8 aa, Artificial Sequence
  28H1 heavy chain CDR3
GWLGNFDY

SEQ ID NO: 148 - protein, 116 aa, Artificial Sequence
  28H1 heavy chain variable region
EVQLLESGGGLVQPGGSLRLSCAASGFTFSSHAMSWVRQAPGKGLEWVSAIWASGEQYYADSVKGRFTISRDNSKNTLYLQMNSLRAQDTAVYYCAKGWLGNFDYWGQGTLVTVSS

SEQ ID NO: 149 - protein, 17 aa, Artificial Sequence
  5E5 light chain CDR1
KSSQSLLNSGDQKNYLT

SEQ ID NO: 150 - protein, 7 aa, Artificial Sequence
  5E5 light chain CDR2
WASTRES

SEQ ID NO: 151 - protein, 9 aa, Artificial Sequence
  5E5 light chain CDR3
QNDYSYPLT

SEQ ID NO: 152 - protein, 113 aa, Artificial Sequence
  5E5 light chain variable region
ELVMTQSPSSLTVTAGEKVTMICKSSQSLLNSGDQKNYLTWYQQKPGQPPKLLIFWASTRESGVPDRFTGSGSGTDFTLTISSVQAEDLAVYYCQNDYSYPLTFGAGTKLELK

SEQ ID NO: 153 - protein, 5 aa, Artificial Sequence
  5E5 heavy chain CDR1
DHAIH

SEQ ID NO: 154 - protein, 17 aa, Artificial Sequence
  5E5 heavy chain CDR2
HFSPGNTDIKYNDKFKG

SEQ ID NO: 155 - protein, 7 aa, Artificial Sequence
  5E5 heavy chain CDR3
STFFFDY

SEQ ID NO: 156 - protein, 116 aa, Artificial Sequence
  5E5 heavy chain variable region
QVQLQQSDAELVKPGSSVKISCKASGYTFTDHAIHWVKQKPEQGLEWIGHFSPGNTDIKYNDKFKGKATLTVDRSSSTAYMQLNSLTSEDSAVYFCKTSTFFFDYWGQGTTLTVSS

SEQ ID NO: 157 - protein, 10 aa, Artificial Sequence
  E-mab light chain CDR1
SASSSISYMY

SEQ ID NO: 158 - protein, 7 aa, Artificial Sequence
  E-mab light chain CDR2
DTSKLAS

SEQ ID NO: 159 - protein, 9 aa, Artificial Sequence
  E-mab light chain CDR3
HQRDSYPWT

SEQ ID NO: 160 - protein, 106 aa, Artificial Sequence
  E-mab light chain variable region
QVVLTQSPVIMSASPGEKVTMTCSASSSISYMYWYQQKPGTSPKRWIYDTSKLASGVPARFSGSGSGTSYSLTISNMEAGDAATYYCHQRDSYPWTFGGGTNLEIK

SEQ ID NO: 161 - protein, 5 aa, Artificial Sequence
  E-mab heavy chain CDR1
KFGVN

SEQ ID NO: 162 - protein, 16 aa, Artificial Sequence
  E-mab heavy chain CDR2
VIWGDGSTSYNSGLIS

SEQ ID NO: 163 - protein, 5 aa, Artificial Sequence
  E-mab heavy chain CDR3
PGGDY

SEQ ID NO: 164 - protein, 113 aa, Artificial Sequence
  E-mab heavy chain variable region
QVQLKESGPDLVAPSQSLSITCTVSGFSLSKFGVNWVRQPPGKGLEWLGVIWGDGSTSYNSGLISRLSISKENSKSQVFLKLNSLQADDTATYYCVKPGGDYWGHGTSVTVSS

SEQ ID NO: 165 - protein, 5 aa, Artificial Sequence
  A-mab light chain CDR1
SYMHW

SEQ ID NO: 166 - protein, 7 aa, Artificial Sequence
  A-mab light chain CDR2
DTSKLAS

SEQ ID NO: 167 - protein, 9 aa, Artificial Sequence
  A-mab light chain CDR3
QQWSKHPLT

SEQ ID NO: 168 - protein, 106 aa, Artificial Sequence
  A-mab light chain variable region
DIELTQSPAIMSASPGEKVTMTCSASSSVSYMHWYQQKSGTSPKRWIYDTSKLASGVPGRFSGSGSGNSYSLTISSVEAEDDATYYCQQWSKHPLTFGSGTKVEIK

SEQ ID NO: 169 - protein, 5 aa, Artificial Sequence
  A-mab heavy chain CDR1
GYTMN

SEQ ID NO: 170 - protein, 17 aa, Artificial Sequence
  A-mab heavy chain CDR2
LITPYNGASSYNQKFRG

SEQ ID NO: 171 - protein, 10 aa, Artificial Sequence
  A-mab heavy chain CDR3
GGYDGRGFDY

SEQ ID NO: 172 - protein, 119 aa, Artificial Sequence
  A-mab heavy chain variable region
QVQLQQSGPELEKPGASVKISCKASGYSFTGYTMNWVKQSHGKSLEWIGLITPYNGASSYNQKFRGKATLTVDKSSSTAYMDLLSLTSEDSAVYFCARGGYDGRGFDYWGSGTPVTVSS

SEQ ID NO: 173 - protein, 133 aa, Artificial Sequence
  husIL2
APTSSSTKKTQLQLEHLLLDLQMILNGINNYKNPKLTRMLTFKFYMPKKATELKHLQCLEEELKPLEEVLNLAQSKNFHFDPRDVVSNINVFVLELKGSETTFMCEYADETATIVEFLNRWITFCQSIISTLT

SEQ ID NO: 174 - protein, 186 aa, Artificial Sequence
  muIFNa4
MARLCAFLMILVMMSYYWSACSLGCDLPHTYNLGNKRALTVLEEMRRLPPLSCLKDRKDFGFPLEKVDNQQIQKAQAILVLRDLTQQILNLFTSKDLSATWNATLLDSFCNDLHQQLNDLKACVMQEPPLTQEDSLLAVRTYFHRITVYLRKKKHSLCAWEVIRAEVWRALSSSTNLLARLSEEKE

SEQ ID NO: 175 - protein, 188 aa, Artificial Sequence
  huIFNa2
MALTFALLVALLVLSCKSSCSVGCDLPQTHSLGSRRTLMLLAQMRRISLFSCLKDRHDFGFPQEEFGNQFQKAETIPVLHEMIQQIFNLFSTKDSSAAWDETLLDKFYTELYQQLNDLEACVIQGVGVTETPLMKEDSILAVRKYFQRITLYLKEKKYSPCAWEVVRAEIMRSFSLSTNLQESLRSKE

SEQ ID NO: 176 - protein, 182 aa, Artificial Sequence
  muIFNb
MNNRWILHAAFLLCFSTTALSINYKQLQLQERTNIRKCQELLEQLNGKINLTYRADFKIPMEMTEKMQKSYTAFAIQEMLQNVFLVFRNNFSSTGWNETIVVRLLDELHQQTVFLKTVLEEKQEERLTWEMSSTALHLKSYYWRVQRYLKLMKYNSYAWMVVRAEIFRNFLIIRRLTRNFQN

SEQ ID NO: 177 - protein, 187 aa, Artificial Sequence
  huIFNb
MTNKCLLQIALLLCFSTTALSMSYNLLGFLQRSSNFQCQKLLWQLNGRLEYCLKDRMNFDIPEEIKQLQQFQKEDAALTIYEMLQNIFAIFRQDSSSTGWNETIVENLLANVYHQINHLKTVLEEKLEKEDFTRGKLMSSLHLKRYYGRILHYLKAKEYSHCAWTIVRVEILRNFYFINRLTGYLRN

SEQ ID NO: 178 - protein, 200 aa, Artificial Sequence
  huIFNL
MAAAWTVVLVTLVLGLAVAGPVPTSKPTTTGKGCHIGRFKSLSPQELASFKKARDALEESLKLKNWSCSSPVFPGNWDLRLLQVRERPVALEAELALTLKVLEAAAGPALEDVLDQPLHTLHHILSQLQACIQPQPTAGPRPRGRLHHWLHRLQEAPKKESAGCLEASVTFNLFRLLTRDLKYVADGNLCLRTSTHPEST

SEQ ID NO: 179 - protein, 160 aa, Artificial Sequence
  huIL10
SPGQGTQSENSCTHFPGNLPNMLRDLRDAFSRVKTFFQMKDQLDNLLLKESLLEDFKGYLGCQALSEMIQFYLEEVMPQAENQDPDIKAHVNSLGENLKTLRLRLRRCHRFLPCENKSKAVEQVKNAFNKLQEKGIYKAMSEFDIFINYIEAYMTMKIRN

SEQ ID NO: 180 - protein, 335 aa, Artificial Sequence
  (huIL10)2
SPGQGTQSENSCTHFPGNLPNMLRDLRDAFSRVKTFFQMKDQLDNLLLKESLLEDFKGYLGCQALSEMIQFYLEEVMPQAENQDPDIKAHVNSLGENLKTLRLRLRRCHRFLPCENKSKAVEQVKNAFNKLQEKGIYKAMSEFDIFINYIEAYMTMKIRNGGGGSGGGGSGGGGSSPGQGTQSENSCTHFPGNLPNMLRDLRDAFSRVKTFFQMKDQLDNLLLKESLLEDFKGYLGCQALSEMIQFYLEEVMPQAENQDPDIKAHVNSLGENLKTLRLRLRRCHRFLPCENKSKAVEQVKNAFNKLQEKGIYKAMSEFDIFINYIEAYMTMKIRN